European Patent Application EP 4 163 297 A1, published April 12, 2023. Title: T CELL ANTIGEN RECEPTOR, MULTIMERIC COMPLEX THEREOF AND PREPARATION METHOD AND USE THEREOF. Applicant: BRISTAR IMMUNOTECH LIMITED, TSINGHUA UNIVERSITY. The sequence listing filed with the application follows.

SEQUENCE LISTING (283 sequences)

SEQ ID NO: 1 - protein, 9 aa, Artificial Sequence
  Epitope
NLVPMVATV

SEQ ID NO: 2 - protein, 9 aa, Artificial Sequence
  Epitope
QYDPVAALF

SEQ ID NO: 3 - protein, 9 aa, Artificial Sequence
  Epitope
ATVQGQNLK

SEQ ID NO: 4 - protein, 6 aa, Artificial Sequence
  CDR
SSNFYA

SEQ ID NO: 5 - protein, 6 aa, Artificial Sequence
  CDR
NSAFQY

SEQ ID NO: 6 - protein, 7 aa, Artificial Sequence
  CDR
TSESDYY

SEQ ID NO: 7 - protein, 6 aa, Artificial Sequence
  CDR
NSMFDY

SEQ ID NO: 8 - protein, 7 aa, Artificial Sequence
  CDR
MTLNGDE

SEQ ID NO: 9 - protein, 6 aa, Artificial Sequence
  CDR
TYSSGN

SEQ ID NO: 10 - protein, 8 aa, Artificial Sequence
  CDR
QEAYKQQN

SEQ ID NO: 11 - protein, 7 aa, Artificial Sequence
  CDR
ISSIKDK

SEQ ID NO: 12 - protein, 9 aa, Artificial Sequence
  CDR
ARNTGNQFY

SEQ ID NO: 13 - protein, 8 aa, Artificial Sequence
  CDR
ASGTYKYI

SEQ ID NO: 14 - protein, 10 aa, Artificial Sequence
  CDR
ATFLTGNQFY

SEQ ID NO: 15 - protein, 8 aa, Artificial Sequence
  CDR
ARYGNKLV

SEQ ID NO: 16 - protein, 14 aa, Artificial Sequence
  CDR
AYRAFYTGANSKLT

SEQ ID NO: 17 - protein, 12 aa, Artificial Sequence
  CDR
AASAWNTGNQFY

SEQ ID NO: 18 - protein, 5 aa, Artificial Sequence
  CDR
MNHEY

SEQ ID NO: 19 - protein, 5 aa, Artificial Sequence
  CDR
SGHDY

SEQ ID NO: 20 - protein, 5 aa, Artificial Sequence
  CDR
SGHVS

SEQ ID NO: 21 - protein, 5 aa, Artificial Sequence
  CDR
SGHDT

SEQ ID NO: 22 - protein, 5 aa, Artificial Sequence
  CDR
SGHRS

SEQ ID NO: 23 - protein, 6 aa, Artificial Sequence
  CDR
SVGAGI

SEQ ID NO: 24 - protein, 6 aa, Artificial Sequence
  CDR
FNNNVP

SEQ ID NO: 25 - protein, 6 aa, Artificial Sequence
  CDR
FQNEAQ

SEQ ID NO: 26 - protein, 6 aa, Artificial Sequence
  CDR
YYEEEE

SEQ ID NO: 27 - protein, 6 aa, Artificial Sequence
  CDR
YFSETQ

SEQ ID NO: 28 - protein, 14 aa, Artificial Sequence
  CDR
ASSFATGVGSYGYT

SEQ ID NO: 29 - protein, 12 aa, Artificial Sequence
  CDR
ASRPLGVGETQY

SEQ ID NO: 30 - protein, 11 aa, Artificial Sequence
  CDR
ASSFSLPYEQY

SEQ ID NO: 31 - protein, 12 aa, Artificial Sequence
  CDR
ASSFYTGQETQY

SEQ ID NO: 32 - protein, 14 aa, Artificial Sequence
  CDR
ASSFFRGEGNQPQH

SEQ ID NO: 33 - protein, 13 aa, Artificial Sequence
  CDR
ASSLAGYKQETQY

SEQ ID NO: 34 - protein, 561 aa, Artificial Sequence
  antigen
MESRGRRCPEMISVLGPISGHVLKAVFSRGDTPVLPHETRLLQTGIHVRVSQPSLILVSQYTPDSTPCHRGDNQLQVQHTYFTGSEVENVSVNVHNPTGRSICPSQEPMSIYVYALPLKMLNIPSINVHHYPSAAERKHRHLPVADAVIHASGKQMWQARLTVSGLAWTRQQNQWKEPDVYYTSAFVFPTKDVALRHVVCAHELVCSMENTRATKMQVIGDQYVKVYLESFCEDVPSGKLFMHVTLGSDVEEDLTMTRNPQPFMRPHERNGFTVLCPKNMIIKPGKISHIMLDVAFTSHEHFGLLCPKSIPGLSISGNLLMNGQQIFLEVQAIRETVELRQYDPVAALFFFDIDLLLQRGPQYSEHPTFTSQYRIQGKLEYRHTWDRHDEGAAQGDDDVWTSGSDSDEELVTTERKTPRVTGGGAMASASTSAGRKRKSASSATACTAGVMTRGRLKAESTVAPEEDTDEDSDNEIHNPAVFTWPPWQAGILARNLVPMVATVQGQNLKYQEFFWDANDIYRIFAELEGVWQPAAQPKRRRHRQDALPGPCIASTPKKHRG

SEQ ID NO: 35 - DNA, 1686 bp, Artificial Sequence
  antigen
atggagtcgcgcggtcgccgttgtcccgaaatgatatccgtactgggtcccatttcggggcacgtgctgaaagccgtgtttagtcgcggcgatacgccggtgctgccgcacgagacgcgactcctgcagacgggtatccacgtacgcgtgagccagccctcgctgatcctggtgtcgcagtacacgcccgactcgacgccatgccaccgcggcgacaatcagctgcaggtgcagcacacgtactttacgggcagcgaggtggagaacgtgtcggtcaacgtgcacaaccccacgggccgaagcatctgccccagccaagagcccatgtcgatctatgtgtacgcgctgccgctcaagatgctgaacatccccagcatcaacgtgcaccactacccgtcggcggccgagcgcaaacaccgacacctgcccgtagccgacgctgttattcacgcgtcgggcaagcagatgtggcaggcgcgtctcacggtctcgggactggcctggacgcgtcagcagaaccagtggaaagagcccgacgtctactacacgtcagcgttcgtgtttcccaccaaggacgtggcactgcggcacgtggtgtgcgcgcacgagctggtttgctccatggagaacacgcgcgcaaccaagatgcaggtgataggtgaccagtacgtcaaggtgtacctggagtccttctgcgaggacgtgccctccggcaagctctttatgcacgtcacgctgggctctgacgtggaagaggacctaacgatgacccgcaacccgcaacccttcatgcgcccccacgagcgcaacggctttacggtgttgtgtcccaaaaatatgataatcaaaccgggcaagatctcgcacatcatgctggatgtggcttttacctcacacgagcattttgggctgctgtgtcccaagagcatcccgggcctgagcatctcaggtaacctgttgatgaacgggcagcaaatcttcctggaggtacaagcgatacgcgagaccgtggaactgcgtcagtacgatcccgtggctgcgctcttctttttcgatatcgacttgttgctgcagcgcgggcctcagtacagcgagcaccccaccttcaccagccagtatcgcatccagggcaagcttgagtaccgacacacctgggaccggcacgacgagggtgccgcccagggcgacgacgacgtctggaccagcggatcggactccgacgaagaactcgtaaccaccgagcgtaagacgccccgcgtcaccggcggcggcgccatggcgagcgcctccacttccgcgggccgcaaacgcaaatcagcatcctcggcgacggcgtgcacggcgggcgttatgacacgcggccgccttaaggccgagtccaccgtcgcgcccgaagaggacaccgacgaggattccgacaacgaaatccacaatccggccgtgttcacctggccgccctggcaggccggcatcctggcccgcaacctggtgcccatggtggctacggttcagggtcagaatctgaagtaccaggagttcttctgggacgccaacgacatctaccgcatcttcgccgaattggaaggcgtatggcagcccgctgcgcaacccaaacgtcgccgccaccggcaagacgccttgcccgggccatgcatcgcctcgacgcccaaaaagcaccgaggttga

SEQ ID NO: 36 - protein, 611 aa, Artificial Sequence
  C22 AA
MSIGLLCCAALSLLWAGPVNAGVTQTPKFQVLKTGQSMTLQCAQDMNHEYMSWYRQDPGMGLRLIHYSVGAGITDQGEVPNGYNVSRSTTEDFPLRLLSAAPSQTSVYFCASSFATGVGSYGYTFGSGTRLTVVEDLKNVFPPEVAVFEPSEAEISHTQKATLVCLATGFFPDHVELSWWVNGKEVHSGVSTDPQPLKEQPALNDSRYCLSSRLRVSATFWQNPRNHFRCQVQFYGLSENDEWTQDRAKPVTQIVSAEAWGRADCGFTSVSYQQGVLSATILYEILLGKATLYAVLVSALVLMAMVKRKDFRRKRSGSGATNFSLLKQAGDVEENPGPMEKNPLAAPLLILWFHLDCVSSILNVEQSPQSLHVQEGDSTNFTCSFPSSNFYALHWYRWETAKSPEALFVMTLNGDEKKKGRISATLNTKEGYSYLYIKGSQPEDSATYLCARNTGNQFYFGTGTSLTVIPNIQNPDPAVYQLRDSKSSDKSVCLFTDFDSQTNVSQSKDSDVYITDKTVLDMRSMDFKSNSAVAWSNKSDFACANAFNNSIIPEDTFFPSPESSCDVKLVEKSFETDTNLNFQNLSVIGFRILLLKVAGFNLLMTLRLWSS

SEQ ID NO: 37 - DNA, 1836 bp, Artificial Sequence
  C22 NT
atgagcatcggcctcctgtgctgtgcagccttgtctctcctgtgggcaggtccagtgaatgctggtgtcactcagaccccaaaattccaggtcctgaagacaggacagagcatgacactgcagtgtgcccaggatatgaaccatgaatacatgtcctggtatcgacaagacccaggcatggggctgaggctgattcattactcagttggtgctggtatcactgaccaaggagaagtccccaatggctacaatgtctccagatcaaccacagaggatttcccgctcaggctgctgtcggctgctccctcccagacatctgtgtacttctgtgccagcagtttcgcgacaggggtggggagctatggctacaccttcggttcggggaccaggttaaccgttgtagaggacctgaaaaacgtgttcccacccgaggtcgctgtgtttgagccatcagaagcagagatctcccacacccaaaaggccacactggtgtgcctggccacaggcttcttccccgaccacgtggagctgagctggtgggtgaatgggaaggaggtgcacagtggggtcagcacagacccgcagcccctcaaggagcagcccgccctcaatgactccagatactgcctgagcagccgcctgagggtctcggccaccttctggcagaacccccgcaaccacttccgctgtcaagtccagttctacgggctctcggagaatgacgagtggacccaggatagggccaaacccgtcacccagatcgtcagcgccgaggcctggggtagagcagactgtggctttacctcggtgtcctaccagcaaggggtcctgtctgccaccatcctctatgagatcctgctagggaaggccaccctgtatgctgtgctggtcagcgcccttgtgttgatggccatggtcaagagaaaggatttccggcggaaacggagcggaagcggagctactaacttcagcctgctgaagcaggctggagacgtggaggagaaccctggacctatggagaagaatcctttggcagccccattactaatcctctggtttcatcttgactgcgtgagcagcatactgaacgtggaacaaagtcctcagtcactgcatgttcaggagggagacagcaccaatttcacctgcagcttcccttccagcaatttttatgccttacactggtacagatgggaaactgcaaaaagccccgaggccttgtttgtaatgactttaaatggggatgaaaagaagaaaggacgaataagtgccactcttaataccaaggagggttacagctatttgtacatcaaaggatcccagcctgaagactcagccacatacctctgtgcccggaacaccggtaaccagttctattttgggacagggacaagtttgacggtcattccaaatatccagaaccctgaccctgccgtgtaccagctgagagactctaaatccagtgacaagtctgtctgcctattcaccgattttgattctcaaacaaatgtgtcacaaagtaaggattctgatgtgtatatcacagacaaaactgtgctagacatgaggtctatggacttcaagagcaacagtgctgtggcctggagcaacaaatctgactttgcatgtgcaaacgccttcaacaacagcattattccagaagacaccttcttccccagcccagaaagttcctgtgatgtcaagctggtcgagaaaagctttgaaacagatacgaacctaaactttcaaaacctgtcagtgattgggttccgaatcctcctcctgaaagtggccgggtttaatctgctcatgacgctgcggctgtggtccagctga

SEQ ID NO: 38 - protein, 608 aa, Artificial Sequence
  C27 AA
MSIGLLCCAALSLLWAGPVNAGVTQTPKFQVLKTGQSMTLQCAQDMNHEYMSWYRQDPGMGLRLIHYSVGAGITDQGEVPNGYNVSRSTTEDFPLRLLSAAPSQTSVYFCASRPLGVGETQYFGPGTRLLVLEDLKNVFPPEVAVFEPSEAEISHTQKATLVCLATGFFPDHVELSWWVNGKEVHSGVSTDPQPLKEQPALNDSRYCLSSRLRVSATFWQNPRNHFRCQVQFYGLSENDEWTQDRAKPVTQIVSAEAWGRADCGFTSVSYQQGVLSATILYEILLGKATLYAVLVSALVLMAMVKRKDFRRKRSGSGATNFSLLKQAGDVEENPGPMEKNPLAAPLLILWFHLDCVSSILNVEQSPQSLHVQEGDSTNFTCSFPSSNFYALHWYRWETAKSPEALFVMTLNGDEKKKGRISATLNTKEGYSYLYIKGSQPEDSATYLCASGTYKYIFGTGTRLKVLANIQNPDPAVYQLRDSKSSDKSVCLFTDFDSQTNVSQSKDSDVYITDKTVLDMRSMDFKSNSAVAWSNKSDFACANAFNNSIIPEDTFFPSPESSCDVKLVEKSFETDTNLNFQNLSVIGFRILLLKVAGFNLLMTLRLWSS

SEQ ID NO: 39 - DNA, 1827 bp, Artificial Sequence
  C27 NT
atgagcatcggcctcctgtgctgtgcagccttgtctctcctgtgggcaggtccagtgaatgctggtgtcactcagaccccaaaattccaggtcctgaagacaggacagagcatgacactgcagtgtgcccaggatatgaaccatgaatacatgtcctggtatcgacaagacccaggcatggggctgaggctgattcattactcagttggtgctggtatcactgaccaaggagaagtccccaatggctacaatgtctccagatcaaccacagaggatttcccgctcaggctgctgtcggctgctccctcccagacatctgtgtacttctgtgccagcagaccactgggggtcggcgagacccagtacttcgggccaggcacgcggctcctggtgctcgaggacctgaaaaacgtgttcccacccgaggtcgctgtgtttgagccatcagaagcagagatctcccacacccaaaaggccacactggtgtgcctggccacaggcttcttccccgaccacgtggagctgagctggtgggtgaatgggaaggaggtgcacagtggggtcagcacagacccgcagcccctcaaggagcagcccgccctcaatgactccagatactgcctgagcagccgcctgagggtctcggccaccttctggcagaacccccgcaaccacttccgctgtcaagtccagttctacgggctctcggagaatgacgagtggacccaggatagggccaaacccgtcacccagatcgtcagcgccgaggcctggggtagagcagactgtggctttacctcggtgtcctaccagcaaggggtcctgtctgccaccatcctctatgagatcctgctagggaaggccaccctgtatgctgtgctggtcagcgcccttgtgttgatggccatggtcaagagaaaggatttccggcggaaacggagcggaagcggagctactaacttcagcctgctgaagcaggctggagacgtggaggagaaccctggacctatggagaagaatcctttggcagccccattactaatcctctggtttcatcttgactgcgtgagcagcatactgaacgtggaacaaagtcctcagtcactgcatgttcaggagggagacagcaccaatttcacctgcagcttcccttccagcaatttttatgccttacactggtacagatgggaaactgcaaaaagccccgaggccttgtttgtaatgactttaaatggggatgaaaagaagaaaggacgaataagtgccactcttaataccaaggagggttacagctatttgtacatcaaaggatcccagcctgaagactcagccacatacctctgtgcttcaggaacctacaaatacatctttggaacaggcaccaggctgaaggttttagcaaatatccagaaccctgaccctgccgtgtaccagctgagagactctaaatccagtgacaagtctgtctgcctattcaccgattttgattctcaaacaaatgtgtcacaaagtaaggattctgatgtgtatatcacagacaaaactgtgctagacatgaggtctatggacttcaagagcaacagtgctgtggcctggagcaacaaatctgactttgcatgtgcaaacgccttcaacaacagcattattccagaagacaccttcttccccagcccagaaagttcctgtgatgtcaagctggtcgagaaaagctttgaaacagatacgaacctaaactttcaaaacctgtcagtgattgggttccgaatcctcctcctgaaagtggccgggtttaatctgctcatgacgctgcggctgtggtccagctga

SEQ ID NO: 40 - protein, 609 aa, Artificial Sequence
  C29 AA
MDSWTFCCVSLCILVAKHTDAGVIQSPRHEVTEMGQEVTLRCKPISGHDYLFWYRQTMMRGLELLIYFNNNVPIDDSGMPEDRFSAKMPNASFSTLKIQPSEPRDSAVYFCASSFSLPYEQYFGPGTRLTVTEDLKNVFPPEVAVFEPSEAEISHTQKATLVCLATGFFPDHVELSWWVNGKEVHSGVSTDPQPLKEQPALNDSRYCLSSRLRVSATFWQNPRNHFRCQVQFYGLSENDEWTQDRAKPVTQIVSAEAWGRADCGFTSVSYQQGVLSATILYEILLGKATLYAVLVSALVLMAMVKRKDFRRKRSGSGATNFSLLKQAGDVEENPGPMMKSLRVLLVILWLQLSWVWSQQKEVEQDPGPLSVPEGAIVSLNCTYSNSAFQYFMWYRQYSRKGPELLMYTYSSGNKEDGRFTAQVDKSSKYISLFIRDSQPSDSATYLCATFLTGNQFYFGTGTSLTVIPNIQNPDPAVYQLRDSKSSDKSVCLFTDFDSQTNVSQSKDSDVYITDKTVLDMRSMDFKSNSAVAWSNKSDFACANAFNNSIIPEDTFFPSPESSCDVKLVEKSFETDTNLNFQNLSVIGFRILLLKVAGFNLLMTLRLWSS

SEQ ID NO: 41 - DNA, 1830 bp, Artificial Sequence
  C29 NT
atggactcctggaccttctgctgtgtgtccctttgcatcctggtagcaaagcacacagatgctggagttatccagtcaccccggcacgaggtgacagagatgggacaagaagtgactctgagatgtaaaccaatttcaggacatgactaccttttctggtacagacagaccatgatgcggggactggagttgctcatttactttaacaacaacgttccgatagatgattcagggatgcccgaggatcgattctcagctaagatgcctaatgcatcattctccactctgaagatccagccctcagaacccagggactcagctgtgtacttctgtgccagcagttttagccttccctacgagcagtacttcgggccgggcaccaggctcacggtcacagaggacctgaaaaacgtgttcccacccgaggtcgctgtgtttgagccatcagaagcagagatctcccacacccaaaaggccacactggtgtgcctggccacaggcttcttccccgaccacgtggagctgagctggtgggtgaatgggaaggaggtgcacagtggggtcagcacagacccgcagcccctcaaggagcagcccgccctcaatgactccagatactgcctgagcagccgcctgagggtctcggccaccttctggcagaacccccgcaaccacttccgctgtcaagtccagttctacgggctctcggagaatgacgagtggacccaggatagggccaaacccgtcacccagatcgtcagcgccgaggcctggggtagagcagactgtggctttacctcggtgtcctaccagcaaggggtcctgtctgccaccatcctctatgagatcctgctagggaaggccaccctgtatgctgtgctggtcagcgcccttgtgttgatggccatggtcaagagaaaggatttccggcggaaacggagcggaagcggagctactaacttcagcctgctgaagcaggctggagacgtggaggagaaccctggacctatgatgaaatccttgagagttttactggtgatcctgtggcttcagttaagctgggtttggagccaacagaaggaggtggagcaggatcctggaccactcagtgttccagagggagccattgtttctctcaactgcacttacagcaacagtgcttttcaatacttcatgtggtacagacagtattccagaaaaggccctgagttgctgatgtacacatactccagtggtaacaaagaagatggaaggtttacagcacaggtcgataaatccagcaagtatatctccttgttcatcagagactcacagcccagtgattcagccacctacctctgtgcaacttttttaaccggtaaccagttctattttgggacagggacaagtttgacggtcattccaaatatccagaaccctgaccctgccgtgtaccagctgagagactctaaatccagtgacaagtctgtctgcctattcaccgattttgattctcaaacaaatgtgtcacaaagtaaggattctgatgtgtatatcacagacaaaactgtgctagacatgaggtctatggacttcaagagcaacagtgctgtggcctggagcaacaaatctgactttgcatgtgcaaacgccttcaacaacagcattattccagaagacaccttcttccccagcccagaaagttcctgtgatgtcaagctggtcgagaaaagctttgaaacagatacgaacctaaactttcaaaacctgtcagtgattgggttccgaatcctcctcctgaaagtggccgggtttaatctgctcatgacgctgcggctgtggtccagctga

SEQ ID NO: 42 - protein, 609 aa, Artificial Sequence
  C30 AA
MGTRLLCWVVLGFLGTDHTGAGVSQSPRYKVAKRGQDVALRCDPISGHVSLFWYQQALGQGPEFLTYFQNEAQLDKSGLPSDRFFAERPEGSVSTLKIQRTQQEDSAVYLCASSFYTGQETQYFGPGTRLLVLEDLKNVFPPEVAVFEPSEAEISHTQKATLVCLATGFFPDHVELSWWVNGKEVHSGVSTDPQPLKEQPALNDSRYCLSSRLRVSATFWQNPRNHFRCQVQFYGLSENDEWTQDRAKPVTQIVSAEAWGRADCGFTSVSYQQGVLSATILYEILLGKATLYAVLVSALVLMAMVKRKDFRRKRSGSGATNFSLLKQAGDVEENPGPMEKNPLAAPLLILWFHLDCVSSILNVEQSPQSLHVQEGDSTNFTCSFPSSNFYALHWYRWETAKSPEALFVMTLNGDEKKKGRISATLNTKEGYSYLYIKGSQPEDSATYLCARYGNKLVFGAGTILRVKSYIQNPDPAVYQLRDSKSSDKSVCLFTDFDSQTNVSQSKDSDVYITDKTVLDMRSMDFKSNSAVAWSNKSDFACANAFNNSIIPEDTFFPSPESSCDVKLVEKSFETDTNLNFQNLSVIGFRILLLKVAGFNLLMTLRLWSS

SEQ ID NO: 43 - DNA, 1830 bp, Artificial Sequence
  C30 NT
atgggcaccaggctcctctgctgggtggtcctgggtttcctagggacagatcacacaggtgctggagtctcccagtcccctaggtacaaagtcgcaaagagaggacaggatgtagctctcaggtgtgatccaatttcgggtcatgtatcccttttttggtaccaacaggccctggggcaggggccagagtttctgacttatttccagaatgaagctcaactagacaaatcggggctgcccagtgatcgcttctttgcagaaaggcctgagggatccgtctccactctgaagatccagcgcacacagcaggaggactccgccgtgtatctctgtgccagcagcttttatacggggcaagagacccagtacttcgggccaggcacgcggctcctggtgctcgaggacctgaaaaacgtgttcccacccgaggtcgctgtgtttgagccatcagaagcagagatctcccacacccaaaaggccacactggtgtgcctggccacaggcttcttccccgaccacgtggagctgagctggtgggtgaatgggaaggaggtgcacagtggggtcagcacagacccgcagcccctcaaggagcagcccgccctcaatgactccagatactgcctgagcagccgcctgagggtctcggccaccttctggcagaacccccgcaaccacttccgctgtcaagtccagttctacgggctctcggagaatgacgagtggacccaggatagggccaaacccgtcacccagatcgtcagcgccgaggcctggggtagagcagactgtggctttacctcggtgtcctaccagcaaggggtcctgtctgccaccatcctctatgagatcctgctagggaaggccaccctgtatgctgtgctggtcagcgcccttgtgttgatggccatggtcaagagaaaggatttccggcggaaacggagcggaagcggagctactaacttcagcctgctgaagcaggctggagacgtggaggagaaccctggacctatggagaagaatcctttggcagccccattactaatcctctggtttcatcttgactgcgtgagcagcatactgaacgtggaacaaagtcctcagtcactgcatgttcaggagggagacagcaccaatttcacctgcagcttcccttccagcaatttttatgccttacactggtacagatgggaaactgcaaaaagccccgaggccttgtttgtaatgactttaaatggggatgaaaagaagaaaggacgaataagtgccactcttaataccaaggagggttacagctatttgtacatcaaaggatcccagcctgaagactcagccacatacctctgtgcccgatatggaaacaagctggtctttggcgcaggaaccattctgagagtcaagtcctatatccagaaccctgaccctgccgtgtaccagctgagagactctaaatccagtgacaagtctgtctgcctattcaccgattttgattctcaaacaaatgtgtcacaaagtaaggattctgatgtgtatatcacagacaaaactgtgctagacatgaggtctatggacttcaagagcaacagtgctgtggcctggagcaacaaatctgactttgcatgtgcaaacgccttcaacaacagcattattccagaagacaccttcttccccagcccagaaagttcctgtgatgtcaagctggtcgagaaaagctttgaaacagatacgaacctaaactttcaaaacctgtcagtgattgggttccgaatcctcctcctgaaagtggccgggtttaatctgctcatgacgctgcggctgtggtccagctga

SEQ ID NO: 44 - protein, 616 aa, Artificial Sequence
  C44 AA
MGPGLLCWALLCLLGAGLVDAGVTQSPTHLIKTRGQQVTLRCSPKSGHDTVSWYQQALGQGPQFIFQYYEEEERQRGNFPDRFSGHQFPNYSSELNVNALLLGDSALYLCASSFFRGEGNQPQHFGDGTRLSILEDLKNVFPPEVAVFEPSEAEISHTQKATLVCLATGFFPDHVELSWWVNGKEVHSGVSTDPQPLKEQPALNDSRYCLSSRLRVSATFWQNPRNHFRCQVQFYGLSENDEWTQDRAKPVTQIVSAEAWGRADCGFTSVSYQQGVLSATILYEILLGKATLYAVLVSALVLMAMVKRKDFRRKRSGSGATNFSLLKQAGDVEENPGPMACPGFLWALVISTCLEFSMAQTVTQSQPEMSVQEAETVTLSCTYDTSESDYYLFWYKQPPSRQMILVIRQEAYKQQNATENRFSVNFQKAAKSFSLKISDSQLGDAAMYFCAYRAFYTGANSKLTFGKGITLSVRPDIQNPDPAVYQLRDSKSSDKSVCLFTDFDSQTNVSQSKDSDVYITDKTVLDMRSMDFKSNSAVAWSNKSDFACANAFNNSIIPEDTFFPSPESSCDVKLVEKSFETDTNLNFQNLSVIGFRILLLKVAGFNLLMTLRLWSS

SEQ ID NO: 45 - DNA, 1851 bp, Artificial Sequence
  C44 NT
atgggccccgggctcctctgctgggcactgctttgtctcctgggagcaggcttagtggacgctggagtcacccaaagtcccacacacctgatcaaaacgagaggacagcaagtgactctgagatgctctcctaagtctgggcatgacactgtgtcctggtaccaacaggccctgggtcaggggccccagtttatctttcagtattatgaggaggaagagagacagagaggcaacttccctgatcgattctcaggtcaccagttccctaactatagctctgagctgaatgtgaacgccttgttgctgggggactcggccctctatctctgtgccagcagctttttccggggcgaggggaatcagccccagcattttggtgatgggactcgactctccatcctagaggacctgaaaaacgtgttcccacccgaggtcgctgtgtttgagccatcagaagcagagatctcccacacccaaaaggccacactggtgtgcctggccacaggcttcttccccgaccacgtggagctgagctggtgggtgaatgggaaggaggtgcacagtggggtcagcacagacccgcagcccctcaaggagcagcccgccctcaatgactccagatactgcctgagcagccgcctgagggtctcggccaccttctggcagaacccccgcaaccacttccgctgtcaagtccagttctacgggctctcggagaatgacgagtggacccaggatagggccaaacccgtcacccagatcgtcagcgccgaggcctggggtagagcagactgtggctttacctcggtgtcctaccagcaaggggtcctgtctgccaccatcctctatgagatcctgctagggaaggccaccctgtatgctgtgctggtcagcgcccttgtgttgatggccatggtcaagagaaaggatttccggcggaaacggagcggaagcggagctactaacttcagcctgctgaagcaggctggagacgtggaggagaaccctggacctatggcatgccctggcttcctgtgggcacttgtgatctccacctgtcttgaatttagcatggctcagacagtcactcagtctcaaccagagatgtctgtgcaggaggcagagaccgtgaccctgagctgcacatatgacaccagtgagagtgattattatttattctggtacaagcagcctcccagcaggcagatgattctcgttattcgccaagaagcttataagcaacagaatgcaacagagaatcgtttctctgtgaacttccagaaagcagccaaatccttcagtctcaagatctcagactcacagctgggggatgccgcgatgtatttctgtgcttatagggccttttatactggagccaatagtaagctgacatttggaaaaggaataactctgagtgttagaccagatatccagaaccctgaccctgccgtgtaccagctgagagactctaaatccagtgacaagtctgtctgcctattcaccgattttgattctcaaacaaatgtgtcacaaagtaaggattctgatgtgtatatcacagacaaaactgtgctagacatgaggtctatggacttcaagagcaacagtgctgtggcctggagcaacaaatctgactttgcatgtgcaaacgccttcaacaacagcattattccagaagacaccttcttccccagcccagaaagttcctgtgatgtcaagctggtcgagaaaagctttgaaacagatacgaacctaaactttcaaaacctgtcagtgattgggttccgaatcctcctcctgaaagtggccgggtttaatctgctcatgacgctgcggctgtggtccagctga

SEQ ID NO: 46 - protein, 617 aa, Artificial Sequence
  C45 AA
MGSRLLCWVLLCLLGAGPVKAGVTQTPRYLIKTRGQQVTLSCSPISGHRSVSWYQQTPGQGLQFLFEYFSETQRNKGNFPGRFSGRQFSNSRSEMNVSTLELGDSALYLCASSLAGYKQETQYFGPGTRLLVLEDLKNVFPPEVAVFEPSEAEISHTQKATLVCLATGFFPDHVELSWWVNGKEVHSGVSTDPQPLKEQPALNDSRYCLSSRLRVSATFWQNPRNHFRCQVQFYGLSENDEWTQDRAKPVTQIVSAEAWGRADCGFTSVSYQQGVLSATILYEILLGKATLYAVLVSALVLMAMVKRKDFRRKRSGSGATNFSLLKQAGDVEENPGPMAMLLGASVLILWLQPDWVNSQQKNDDQQVKQNSPSLSVQEGRISILNCDYTNSMFDYFLWYKKYPAEGPTFLISISSIKDKNEDGRFTVFLNKSAKHLSLHIVPSQPGDSAVYFCAASAWNTGNQFYFGTGTSLTVIPNIQNPDPAVYQLRDSKSSDKSVCLFTDFDSQTNVSQSKDSDVYITDKTVLDMRSMDFKSNSAVAWSNKSDFACANAFNNSIIPEDTFFPSPESSCDVKLVEKSFETDTNLNFQNLSVIGFRILLLKVAGFNLLMTLRLWSS

SEQ ID NO: 47 - DNA, 1854 bp, Artificial Sequence
  C45 NT
atgggctccaggctgctctgttgggtgctgctttgtctcctgggagcaggcccagtaaaggctggagtcactcaaactccaagatatctgatcaaaacgagaggacagcaagtgacactgagctgctcccctatctctgggcataggagtgtatcctggtaccaacagaccccaggacagggccttcagttcctctttgaatacttcagtgagacacagagaaacaaaggaaacttccctggtcgattctcagggcgccagttctctaactctcgctctgagatgaatgtgagcaccttggagctgggggactcggccctttatctttgcgccagcagcttggcgggatacaagcaagagacccagtacttcgggccaggcacgcggctcctggtgctcgaggacctgaaaaacgtgttcccacccgaggtcgctgtgtttgagccatcagaagcagagatctcccacacccaaaaggccacactggtgtgcctggccacaggcttcttccccgaccacgtggagctgagctggtgggtgaatgggaaggaggtgcacagtggggtcagcacagacccgcagcccctcaaggagcagcccgccctcaatgactccagatactgcctgagcagccgcctgagggtctcggccaccttctggcagaacccccgcaaccacttccgctgtcaagtccagttctacgggctctcggagaatgacgagtggacccaggatagggccaaacccgtcacccagatcgtcagcgccgaggcctggggtagagcagactgtggctttacctcggtgtcctaccagcaaggggtcctgtctgccaccatcctctatgagatcctgctagggaaggccaccctgtatgctgtgctggtcagcgcccttgtgttgatggccatggtcaagagaaaggatttccggcggaaacggagcggaagcggagctactaacttcagcctgctgaagcaggctggagacgtggaggagaaccctggacctatggccatgctcctgggggcatcagtgctgattctgtggcttcagccagactgggtaaacagtcaacagaagaatgatgaccagcaagttaagcaaaattcaccatccctgagcgtccaggaaggaagaatttctattctgaactgtgactatactaacagcatgtttgattatttcctatggtacaaaaaataccctgctgaaggtcctacattcctgatatctataagttccattaaggataaaaatgaagatggaagattcactgttttcttaaacaaaagtgccaagcacctctctctgcacattgtgccctcccagcctggagactctgcagtgtacttctgtgcagcaagcgcgtggaacaccggtaaccagttctattttgggacagggacaagtttgacggtcattccaaatatccagaaccctgaccctgccgtgtaccagctgagagactctaaatccagtgacaagtctgtctgcctattcaccgattttgattctcaaacaaatgtgtcacaaagtaaggattctgatgtgtatatcacagacaaaactgtgctagacatgaggtctatggacttcaagagcaacagtgctgtggcctggagcaacaaatctgactttgcatgtgcaaacgccttcaacaacagcattattccagaagacaccttcttccccagcccagaaagttcctgtgatgtcaagctggtcgagaaaagctttgaaacagatacgaacctaaactttcaaaacctgtcagtgattgggttccgaatcctcctcctgaaagtggccgggtttaatctgctcatgacgctgcggctgtggtccagctga

SEQ ID NO: 48 - protein, 294 aa, Artificial Sequence
  A0201-aa
MGSHSMRYFFTSVSRPGRGEPRFIAVGYVDDTQFVRFDSDAASQRMEPRAPWIEQEGPEYWDGETRKVKAHSQTHRVDLGTLRGYYNQSEAGSHTVQRMYGCDVGSDWRFLRGYHQYAYDGKDYIALKEDLRSWTAADMAAQTTKHKWEAAHVAEQLRAYLEGTCVEWLRRYLENGKETLQRTDAPKTHMTHHAVSDHEATLRCWALSFYPAEITLTWQRDGEDQTQDTELVETRPAGDGTFQKWVAVVVPSGQEQRYTCHVQHEGLPKPLTLRWEPGSGLNDIFEAQKIEWHE

SEQ ID NO: 49 - DNA, 885 bp, Artificial Sequence
  A0201-DNA
atgggcagccatagcatgcgttacttcttcaccagcgttagtcgccccggtcgcggtgaaccgcgctttatcgcagtgggttacgttgacgacacccagtttgtgcgttttgacagcgatgccgcaagccagcgtatggaaccgcgtgccccgtggattgaacaagaaggcccggaatactgggatggcgaaacccgcaaagttaaagcccacagccagacccatcgcgtggatctgggtactttacgtggctactataaccagagcgaagccggtagccataccgtgcagcgcatgtatggctgtgatgtgggcagtgattggcgctttctgcgcggctatcatcagtacgcctatgacggcaaggactacatcgctttaaaagaagatttacgtagttggaccgccgccgatatggcagcccagaccaccaaacataaatgggaagccgcccatgtggcagagcagctgcgcgcatatctggaaggcacatgcgtggaatggctgcgtcgctatctggagaacggcaaagaaactttacagcgcaccgacgcaccgaaaacccatatgacccaccatgccgtgagtgaccatgaagccactttacgctgttgggctttaagcttctatccggccgaaattactttaacttggcagcgcgatggtgaagaccagacccaagataccgagctggtggaaacccgtccggctggtgatggcacctttcagaaatgggtggccgttgtggtgccgagcggtcaagaacagcgctatacttgtcatgtgcagcatgagggcttaccgaaaccgctgactttacgctgggaaccgggatccggtttgaacgacatcttcgaagctcagaaaatcgaatggcacgaataa

SEQ ID NO: 50 - protein, 294 aa, Artificial Sequence
  A2402-aa
MGSHSMRYFSTSVSRPGRGEPRFIAVGYVDDTQFVRFDSDAASQRMEPRAPWIEQEGPEYWDEETGKVKAHSQTDRENLRIALRYYNQSEAGSHTLQMMFGCDVGSDGRFLRGYHQYAYDGKDYIALKEDLRSWTAADMAAQITKRKWEAAHVAEQQRAYLEGTCVDGLRRYLENGKETLQRTDPPKTHMTHHPISDHEATLRCWALGFYPAEITLTWQRDGEDQTQDTELVETRPAGDGTFQKWVAVVVPSGEEQRYTCHVQHEGLPKPLTLRWEPGSGLNDIFEAQKIEWHE

SEQ ID NO: 51 - DNA, 885 bp, Artificial Sequence
  A2402-DNA
atgggcagccacagtatgcgctacttcagcaccagcgttagtcgcccgggtcgtggtgaaccgcgttttatcgcagtgggctatgtggacgatacccagttcgttcgcttcgacagtgatgccgcaagtcagcgcatggaaccgcgtgccccgtggatcgaacaggaaggcccggaatactgggatgaggaaaccggcaaggtgaaagcacacagccagaccgaccgtgaaaacctgcgcattgccctgcgctattacaatcagagcgaagccggcagccacaccctgcagatgatgtttggttgcgatgtgggcagtgatggtcgctttctgcgcggctatcaccagtacgcctacgacggcaaggattatatcgccctgaaagaagacctgcgtagctggaccgcagccgatatggccgcccagattaccaaacgcaaatgggaggccgcacatgttgccgaacaacagcgcgcatatctggaaggtacctgtgtggatggtctgcgtcgctatctggaaaacggcaaagaaaccctgcagcgcaccgatcctccgaaaacccacatgacccaccacccgatcagcgaccatgaagccacactgcgttgctgggccctgggcttttacccggccgaaatcaccctgacctggcagcgcgatggcgaagatcagacccaggacaccgaactggtggaaacccgtccggcaggtgatggcacctttcagaaatgggtggcagtggttgtgccgagcggcgaagaacagcgttatacctgccatgtgcagcacgaaggtctgccgaaaccgctgaccctgcgctgggaacctggatccggtttgaacgacatcttcgaagctcagaaaatcgaatggcacgaataa

SEQ ID NO: 52 - protein, 294 aa, Artificial Sequence
  A1101-aa
MGSHSMRYFYTSVSRPGRGEPRFIAVGYVDDTQFVRFDSDAASQRMEPRAPWIEQEGPEYWDQETRNVKAQSQTDRVDLGTLRGYYNQSEDGSHTIQIMYGCDVGPDGRFLRGYRQDAYDGKDYIALNEDLRSWTAADMAAQITKRKWEAAHAAEQQRAYLEGRCVEWLRRYLENGKETLQRTDPPKTHMTHHPISDHEATLRCWALGFYPAEITLTWQRDGEDQTQDTELVETRPAGDGTFQKWVAVVVPSGEEQRYTCHVQHEGLPKPLTLRWELGSGLNDIFEAQKIEWHE

SEQ ID NO: 53 - DNA, 885 bp, Artificial Sequence
  A1101-DNA
atgggtagccatagcatgcgctacttctataccagcgtgagtcgtccgggccgtggtgaacctcgctttattgccgtgggctatgtggatgacacccagttcgtgcgctttgatagcgatgccgcaagtcagcgcatggaaccgcgtgccccgtggattgaacaagaaggcccggaatattgggaccaagaaacacgcaacgttaaggcccagagccagacagatcgtgtggatctgggtacactgcgcggctattacaatcagagcgaggatggcagccacaccattcagatcatgtacggctgcgatgttggtccggacggtcgctttttacgtggctaccgtcaagatgcctatgatggcaaggactatatcgctttaaacgaggatctgcgcagttggaccgcagccgatatggccgcacagatcaccaaacgcaaatgggaagcagcacacgccgccgagcagcaacgtgcatatttagaaggtcgttgcgtggaatggctgcgccgctatctggagaatggcaaagaaactttacagcgtaccgatccgccgaaaacccatatgacccatcacccgatcagcgatcatgaggccactttacgttgttgggcactgggcttttatccggcagaaatcactttaacttggcagcgcgatggtgaagatcagacccaagataccgaactggtggaaacccgccccgctggtgatggcacctttcagaaatgggttgcagtggttgtgccgagcggcgaggaacagcgttacacttgtcacgttcagcatgaaggtttaccgaaaccgctgactttacgttgggaactgggatccggtttgaacgacatcttcgaagctcagaaaatcgaatggcacgaataa

SEQ ID NO: 54 - protein, 101 aa, Artificial Sequence
  b2m-aa
MAIQRTPKIQVYSRHPAENGKSNFLNCYVSGFHPSDIEVDLLKNGERIEKVEHSDLSFSKDWSFYLLYYTEFTPTEKDEYACRVNHVTLSQPKIVKWDRDM

SEQ ID NO: 55 - DNA, 306 bp, Artificial Sequence
  b2m-DNA
atggcaatccagcgtactccaaagattcaggtttactcacgtcatccagcagagaatggaaagtcaaatttcctgaattgctatgtgtctgggtttcatccatccgacattgaagttgacttactgaagaatggagagagaattgaaaaagtggagcattcagacttgtctttcagcaaggactggtctttctatctcttgtactacactgaattcacccccactgaaaaagatgagtatgcctgccgtgtgaaccatgtgactttgtcacagcccaagatagttaagtgggatcgagacatgtaa

SEQ ID NO: 56 - DNA, 21 bp, Artificial Sequence
  Primer
atggatacctggctcgtatgc

SEQ ID NO: 57 - DNA, 18 bp, Artificial Sequence
  Primer
atgggctgcaggctcctc

SEQ ID NO: 58 - DNA, 18 bp, Artificial Sequence
  Primer
atgggctgcaggctgctc

SEQ ID NO: 59 - DNA, 19 bp, Artificial Sequence
  Primer
atgggctccaggctgctct

SEQ ID NO: 60 - DNA, 14 bp, Artificial Sequence
  Primer
atgggccccgggct

SEQ ID NO: 61 - DNA, 17 bp, Artificial Sequence
  Primer
atgggccctgggctcct

SEQ ID NO: 62 - DNA, 19 bp, Artificial Sequence
  Primer
atgggacccaggctcctct

SEQ ID NO: 63 - DNA, 20 bp, Artificial Sequence
  Primer
atgagcatcgggctcctgtg

SEQ ID NO: 64 - DNA, 18 bp, Artificial Sequence
  Primer
atgagcctcgggctcctg

SEQ ID NO: 65 - DNA, 21 bp, Artificial Sequence
  Primer
atgagaatcaggctcctgtgc

SEQ ID NO: 66 - DNA, 20 bp, Artificial Sequence
  Primer
atgagcatcggcctcctgtg

SEQ ID NO: 67 - DNA, 20 bp, Artificial Sequence
  Primer
atgagcatcagcctcctgtg

SEQ ID NO: 68 - DNA, 20 bp, Artificial Sequence
  Primer
atgggcacaaggctcctctg

SEQ ID NO: 69 - DNA, 18 bp, Artificial Sequence
  Primer
atgggcaccaggctcctc

SEQ ID NO: 70 - DNA, 21 bp, Artificial Sequence
  Primer
atgggcaccagtctcctatgc

SEQ ID NO: 71 - DNA, 23 bp, Artificial Sequence
  Primer
atgggtaccagtctcctatgctg

SEQ ID NO: 72 - DNA, 18 bp, Artificial Sequence
  Primer
atgggcaccagcctcctc

SEQ ID NO: 73 - DNA, 20 bp, Artificial Sequence
  Primer
atgggcttcaggctcctctg

SEQ ID NO: 74 - DNA, 21 bp, Artificial Sequence
  Primer
atgggcacgaggctcttcttc

SEQ ID NO: 75 - DNA, 21 bp, Artificial Sequence
  Primer
atgggcaccaggctcttcttc

SEQ ID NO: 76 - DNA, 21 bp, Artificial Sequence
  Primer
atgggcacaaggttgttcttc

SEQ ID NO: 77 - DNA, 21 bp, Artificial Sequence
  Primer
atgagcaccaggcttctctgc

SEQ ID NO: 78 - DNA, 20 bp, Artificial Sequence
  Primer
atgggtaccaggctcctctg

SEQ ID NO: 79 - DNA, 22 bp, Artificial Sequence
  Primer
atggactcctggaccttctgct

SEQ ID NO: 80 - DNA, 20 bp, Artificial Sequence
  Primer
atggactcctggaccctctg

SEQ ID NO: 81 - DNA, 18 bp, Artificial Sequence
  Primer
atggccaccaggctcctc

SEQ ID NO: 82 - DNA, 22 bp, Artificial Sequence
  Primer
atgcttagtcctgacctgcctg

SEQ ID NO: 83 - DNA, 22 bp, Artificial Sequence
  Primer
atggtttccaggcttctcagtt

SEQ ID NO: 84 - DNA, 19 bp, Artificial Sequence
  Primer
atgggtcctgggcttctcc

SEQ ID NO: 85 - DNA, 22 bp, Artificial Sequence
  Primer
atgagcccaatattcacctgca

SEQ ID NO: 86 - DNA, 22 bp, Artificial Sequence
  Primer
atggatatctggctcctctgct

SEQ ID NO: 87 - DNA, 23 bp, Artificial Sequence
  Primer
atggacaccagagtactctgctg

SEQ ID NO: 88 - DNA, 20 bp, Artificial Sequence
  Primer
atgagcaaccaggtgctctg

SEQ ID NO: 89 - DNA, 19 bp, Artificial Sequence
  Primer
atgctgctgcttctgctgc

SEQ ID NO: 90 - DNA, 21 bp, Artificial Sequence
  Primer
atggcctccctgctcttcttc

SEQ ID NO: 91 - DNA, 24 bp, Artificial Sequence
  Primer
atgactatcaggctcctctgctac

SEQ ID NO: 92 - DNA, 16 bp, Artificial Sequence
  Primer
atgggcccccagctcc

SEQ ID NO: 93 - DNA, 22 bp, Artificial Sequence
  Primer
atgggaatcaggctcctctgtc

SEQ ID NO: 94 - DNA, 24 bp, Artificial Sequence
  Primer
atgctgagtcttctgctccttctc

SEQ ID NO: 95 - DNA, 20 bp, Artificial Sequence
  Primer
atgctctgctctctccttgc

SEQ ID NO: 96 - DNA, 22 bp, Artificial Sequence
  Primer
tcactctgaagatccggtccac

SEQ ID NO: 97 - DNA, 22 bp, Artificial Sequence
  Primer
cttcacatcaattccctggagc

SEQ ID NO: 98 - DNA, 19 bp, Artificial Sequence
  Primer
cacctgaatgccccaacag

SEQ ID NO: 99 - DNA, 21 bp, Artificial Sequence
  Primer
agtcgcttctcacctgaatgc

SEQ ID NO: 100 - DNA, 24 bp, Artificial Sequence
  Primer
gagatgaatgtgagcaccttggag

SEQ ID NO: 101 - DNA, 24 bp, Artificial Sequence
  Primer
gagatgaatgtgagtgccttggag

SEQ ID NO: 102 - DNA, 22 bp, Artificial Sequence
  Primer
gctctgagctgaatgtgaacgc

SEQ ID NO: 103 - DNA, 22 bp, Artificial Sequence
  Primer
gaagtccccaatggctacaatg

SEQ ID NO: 104 - DNA, 21 bp, Artificial Sequence
  Primer
aggtccctgatggctacaatg

SEQ ID NO: 105 - DNA, 20 bp, Artificial Sequence
  Primer
tggcgtctgctgtaccctct

SEQ ID NO: 106 - DNA, 20 bp, Artificial Sequence
  Primer
acagaggatttcccgctcag

SEQ ID NO: 107 - DNA, 20 bp, Artificial Sequence
  Primer
cccctcaagctggagtcagc

SEQ ID NO: 108 - DNA, 23 bp, Artificial Sequence
  Primer
acacagaggatttcccactcagg

SEQ ID NO: 109 - DNA, 22 bp, Artificial Sequence
  Primer
ttctctgcacagaggtctgagg

SEQ ID NO: 110 - DNA, 20 bp, Artificial Sequence
  Primer
gctgcccagtgatcgcttct

SEQ ID NO: 111 - DNA, 22 bp, Artificial Sequence
  Primer
actctgaagatccagcgcacag

SEQ ID NO: 112 - DNA, 23 bp, Artificial Sequence
  Primer
cgtctccactctgaagatccagc

SEQ ID NO: 113 - DNA, 20 bp, Artificial Sequence
  Primer
ggcctgagggatccatctcc

SEQ ID NO: 114 - DNA, 20 bp, Artificial Sequence
  Primer
ggctgctcagtgatcggttc

SEQ ID NO: 115 - DNA, 22 bp, Artificial Sequence
  Primer
gaacgattctccgcacaacagt

SEQ ID NO: 116 - DNA, 24 bp, Artificial Sequence
  Primer
acaaaggagaagtctcagatggct

SEQ ID NO: 117 - DNA, 22 bp, Artificial Sequence
  Primer
ccctcactctggagtcagctac

SEQ ID NO: 118 - DNA, 21 bp, Artificial Sequence
  Primer
cctcactctggagtccgctac

SEQ ID NO: 119 - DNA, 24 bp, Artificial Sequence
  Primer
gcagagaggctcaaaggagtagac

SEQ ID NO: 120 - DNA, 20 bp, Artificial Sequence
  Primer
atccagccctcagaacccag

SEQ ID NO: 121 - DNA, 25 bp, Artificial Sequence
  Primer
atcattctgaactgaacatgagctc

SEQ ID NO: 122 - DNA, 25 bp, Artificial Sequence
  Primer
tggagggacgtattctactctgaag

SEQ ID NO: 123 - DNA, 24 bp, Artificial Sequence
  Primer
gacacccctgataacttccaatcc

SEQ ID NO: 124 - DNA, 20 bp, Artificial Sequence
  Primer
tgcctcccaaattcaccctg

SEQ ID NO: 125 - DNA, 17 bp, Artificial Sequence
  Primer
catcccgcagagccgag

SEQ ID NO: 126 - DNA, 21 bp, Artificial Sequence
  Primer
gcaggtagtgcgaggagattc

SEQ ID NO: 127 - DNA, 20 bp, Artificial Sequence
  Primer
ctgtgacatcggcccaaaag

SEQ ID NO: 128 - DNA, 20 bp, Artificial Sequence
  Primer
acagtgaccagtgcccatcc

SEQ ID NO: 129 - DNA, 19 bp, Artificial Sequence
  Primer
caatgccccaagaacgcac

SEQ ID NO: 130 - DNA, 21 bp, Artificial Sequence
  Primer
tagagtctgccatccccaacc

SEQ ID NO: 131 - DNA, 21 bp, Artificial Sequence
  Primer
gacggagcattttcccctgac

SEQ ID NO: 132 - DNA, 20 bp, Artificial Sequence
  Primer
gccagcaccaaccagacatc

SEQ ID NO: 133 - DNA, 20 bp, Artificial Sequence
  Primer
ctgatcctggagtcgcccag

SEQ ID NO: 134 - DNA, 20 bp, Artificial Sequence
  Primer
atcagccgcccaaacctaac

SEQ ID NO: 135 - DNA, 24 bp, Artificial Sequence
  Primer
cggcagttcatcctgagttctaag

SEQ ID NO: 136 - DNA, 23 bp, Artificial Sequence
  Primer
tcaggcagtatctggagtcattg

SEQ ID NO: 137 - DNA, 20 bp, Artificial Sequence
  Primer
gcacctccttcccattcacc

SEQ ID NO: 138 - DNA, 22 bp, Artificial Sequence
  Primer
gcttctgatggctcaaacacag

SEQ ID NO: 139 - DNA, 20 bp, Artificial Sequence
  Primer
cgaccagcttgacatcacag

SEQ ID NO: 140 - DNA, 25 bp, Artificial Sequence
  Primer
gttgctcttgaagtccatagacctc

SEQ ID NO: 141 - DNA, 20 bp, Artificial Sequence
  Primer
cagggtcagggttctggata

SEQ ID NO: 142 - DNA, 22 bp, Artificial Sequence
  Primer
atgtggggagctttccttctct

SEQ ID NO: 143 - DNA, 25 bp, Artificial Sequence
  Primer
atgtggggagttttccttctttatg

SEQ ID NO: 144 - DNA, 21 bp, Artificial Sequence
  Primer
atggctttgcagagcactctg

SEQ ID NO: 145 - DNA, 20 bp, Artificial Sequence
  Primer
atggcctctgcacccatctc

SEQ ID NO: 146 - DNA, 20 bp, Artificial Sequence
  Primer
atgaggcaagtggcgagagt

SEQ ID NO: 147 - DNA, 24 bp, Artificial Sequence
  Primer
atgaagacatttgctggattttcg

SEQ ID NO: 148 - DNA, 22 bp, Artificial Sequence
  Primer
atggagtcattcctgggaggtg

SEQ ID NO: 149 - DNA, 22 bp, Artificial Sequence
  Primer
atggagaagatgcggagacctg

SEQ ID NO: 150 - DNA, 22 bp, Artificial Sequence
  Primer
atgctcctgttgctcataccag

SEQ ID NO: 151 - DNA, 19 bp, Artificial Sequence
  Primer
atgctcctgctgctcgtcc

SEQ ID NO: 152 - DNA, 21 bp, Artificial Sequence
  Primer
atgctcctggagcttatccca

SEQ ID NO: 153 - DNA, 24 bp, Artificial Sequence
  Primer
atgctcttagtggtcattctgctg

SEQ ID NO: 154 - DNA, 23 bp, Artificial Sequence
  Primer
atgaattcttctccaggaccagc

SEQ ID NO: 155 - DNA, 28 bp, Artificial Sequence
  Primer
atgaactattctccaggcttagtatctc

SEQ ID NO: 156 - DNA, 24 bp, Artificial Sequence
  Primer
atgaaaaagcatctgacgaccttc

SEQ ID NO: 157 - DNA, 27 bp, Artificial Sequence
  Primer
atgatatccttgagagttttactggtg

SEQ ID NO: 158 - DNA, 30 bp, Artificial Sequence
  Primer
atgaaatccttgagagttttactagtgatc

SEQ ID NO: 159 - DNA, 28 bp, Artificial Sequence
  Primer
atgatgaaatccttgagagttttactgg

SEQ ID NO: 160 - DNA, 26 bp, Artificial Sequence
  Primer
atgacatccattcgagctgtatttat

SEQ ID NO: 161 - DNA, 19 bp, Artificial Sequence
  Primer
atggcaggcattcgagctt

SEQ ID NO: 162 - DNA, 24 bp, Artificial Sequence
  Primer
atgtcactttctagcctgctgaag

SEQ ID NO: 163 - DNA, 22 bp, Artificial Sequence
  Primer
atgaagcccaccctcatctcag

SEQ ID NO: 164 - DNA, 23 bp, Artificial Sequence
  Primer
atggaaactctcctgggagtgtc

SEQ ID NO: 165 - DNA, 22 bp, Artificial Sequence
  Primer
atgctgtctgcttcctgctcag

SEQ ID NO: 166 - DNA, 19 bp, Artificial Sequence
  Primer
atgctgactgccagcctgt

SEQ ID NO: 167 - DNA, 23 bp, Artificial Sequence
  Primer
atggagaaaatgttggagtgtgc

SEQ ID NO: 168 - DNA, 20 bp, Artificial Sequence
  Primer
atggagaccctcttgggcct

SEQ ID NO: 169 - DNA, 24 bp, Artificial Sequence
  Primer
atgaagaggatattgggagctctg

SEQ ID NO: 170 - DNA, 25 bp, Artificial Sequence
  Primer
atggacaagatcttaggagcatcat

SEQ ID NO: 171 - DNA, 20 bp, Artificial Sequence
  Primer
atgctgttctccagcctgct

SEQ ID NO: 172 - DNA, 22 bp, Artificial Sequence
  Primer
atggagaagaatcctttggcag

SEQ ID NO: 173 - DNA, 25 bp, Artificial Sequence
  Primer
atgctactcatcacatcaatgttgg

SEQ ID NO: 174 - DNA, 23 bp, Artificial Sequence
  Primer
atgaggctggtggcaagagtaac

SEQ ID NO: 175 - DNA, 25 bp, Artificial Sequence
  Primer
atgaagttggtgacaagcattactg

SEQ ID NO: 176 - DNA, 23 bp, Artificial Sequence
  Primer
atggtcctgaaattctccgtgtc

SEQ ID NO: 177 - DNA, 17 bp, Artificial Sequence
  Primer
atggccatgctcctggg

SEQ ID NO: 178 - DNA, 23 bp, Artificial Sequence
  Primer
atggagactctcctgaaagtgct

SEQ ID NO: 179 - DNA, 25 bp, Artificial Sequence
  Primer
atggagactgttctgcaagtactcc

SEQ ID NO: 180 - DNA, 28 bp, Artificial Sequence
  Primer
atgctccttgaacatttattaataatct

SEQ ID NO: 181 - DNA, 25 bp, Artificial Sequence
  Primer
atgatgaagtgtccacaggctttac

SEQ ID NO: 182 - DNA, 23 bp, Artificial Sequence
  Primer
atgacacgagttagcttgctgtg

SEQ ID NO: 183 - DNA, 18 bp, Artificial Sequence
  Primer
atggcatgccctggcttc

SEQ ID NO: 184 - DNA, 27 bp, Artificial Sequence
  Primer
atgaagaagctactagcaatgattctg

SEQ ID NO: 185 - DNA, 28 bp, Artificial Sequence
  Primer
atgaactcctctctggactttctaattc

SEQ ID NO: 186 - DNA, 20 bp, Artificial Sequence
  Primer
atggtgaagatccggcaatt

SEQ ID NO: 187 - DNA, 26 bp, Artificial Sequence
  Primer
tccttagtcgctctgatagttatggt

SEQ ID NO: 188 - DNA, 27 bp, Artificial Sequence
  Primer
tttcttcattccttagtcggtctaaag

SEQ ID NO: 189 - DNA, 22 bp, Artificial Sequence
  Primer
ctcttcatcgctgctcatcctc

SEQ ID NO: 190 - DNA, 20 bp, Artificial Sequence
  Primer
gccaaacctccttccacctg

SEQ ID NO: 191 - DNA, 20 bp, Artificial Sequence
  Primer
cctgccgacagaaagtccag

SEQ ID NO: 192 - DNA, 20 bp, Artificial Sequence
  Primer
cgcattgcagacacccagac

SEQ ID NO: 193 - DNA, 26 bp, Artificial Sequence
  Primer
ttgataccacccttaaacagagtttg

SEQ ID NO: 194 - DNA, 25 bp, Artificial Sequence
  Primer
attactgaagaatggaagcagcttg

SEQ ID NO: 195 - DNA, 25 bp, Artificial Sequence
  Primer
tcctttaatctgaggaaaccctctg

SEQ ID NO: 196 - DNA, 22 bp, Artificial Sequence
  Primer
gtgaaacctccttccacctgac

SEQ ID NO: 197 - DNA, 24 bp, Artificial Sequence
  Primer
aggctttgaggctgaatttaagag

SEQ ID NO: 198 - DNA, 27 bp, Artificial Sequence
  Primer
ggctgaatttaacaagagtcaaacttc

SEQ ID NO: 199 - DNA, 22 bp, Artificial Sequence
  Primer
gagcgaaacctccttctacctg

SEQ ID NO: 200 - DNA, 23 bp, Artificial Sequence
  Primer
aaaccacttctttccacttggag

SEQ ID NO: 201 - DNA, 23 bp, Artificial Sequence
  Primer
caaagcaaagctctctgcacatc

SEQ ID NO: 202 - DNA, 22 bp, Artificial Sequence
  Primer
cagtgattcagccacctacctc

SEQ ID NO: 203 - DNA, 26 bp, Artificial Sequence
  Primer
cgaattgctgttacattgaacaagac

SEQ ID NO: 204 - DNA, 23 bp, Artificial Sequence
  Primer
ttgcagctactcaacctggagac

SEQ ID NO: 205 - DNA, 21 bp, Artificial Sequence
  Primer
atccgccaaccttgtcatctc

SEQ ID NO: 206 - DNA, 21 bp, Artificial Sequence
  Primer
aaggcgagacatctttccacc

SEQ ID NO: 207 - DNA, 26 bp, Artificial Sequence
  Primer
agattaagagtcacgcttgacacttc

SEQ ID NO: 208 - DNA, 26 bp, Artificial Sequence
  Primer
gccagtcctatcaagagtgacagttc

SEQ ID NO: 209 - DNA, 23 bp, Artificial Sequence
  Primer
caacttcaccatcacagcctcac

SEQ ID NO: 210 - DNA, 22 bp, Artificial Sequence
  Primer
cacatcacagcccctaaacctg

SEQ ID NO: 211 - DNA, 22 bp, Artificial Sequence
  Primer
tggaagacttaatgcctcgctg

SEQ ID NO: 212 - DNA, 21 bp, Artificial Sequence
  Primer
tgtcgctacggaacgctacag

SEQ ID NO: 213 - DNA, 25 bp, Artificial Sequence
  Primer
cttcaataaaagtgccaagcagttc

SEQ ID NO: 214 - DNA, 25 bp, Artificial Sequence
  Primer
aaaaagtggtcgctattctgtcaac

SEQ ID NO: 215 - DNA, 24 bp, Artificial Sequence
  Primer
gaagaaaggacgaataagtgccac

SEQ ID NO: 216 - DNA, 22 bp, Artificial Sequence
  Primer
acatcacagccacccagactac

SEQ ID NO: 217 - DNA, 24 bp, Artificial Sequence
  Primer
cacagaagacagaaagtccagcac

SEQ ID NO: 218 - DNA, 23 bp, Artificial Sequence
  Primer
gcaatcgctgaagacagaaagtc

SEQ ID NO: 219 - DNA, 25 bp, Artificial Sequence
  Primer
gaaaggacagttctctccacatcac

SEQ ID NO: 220 - DNA, 22 bp, Artificial Sequence
  Primer
aaaagtgccaagcacctctctc

SEQ ID NO: 221 - DNA, 22 bp, Artificial Sequence
  Primer
gcaaagctccctgtaccttacg

SEQ ID NO: 222 - DNA, 25 bp, Artificial Sequence
  Primer
aaagataactgccaagttggatgag

SEQ ID NO: 223 - DNA, 26 bp, Artificial Sequence
  Primer
cttcctgaatatctcagcatccatac

SEQ ID NO: 224 - DNA, 22 bp, Artificial Sequence
  Primer
gcatcctgaacatcacagccac

SEQ ID NO: 225 - DNA, 25 bp, Artificial Sequence
  Primer
gaatcgtttctctgtgaacttccag

SEQ ID NO: 226 - DNA, 21 bp, Artificial Sequence
  Primer
tctcagcaccctccacatcac

SEQ ID NO: 227 - DNA, 24 bp, Artificial Sequence
  Primer
caggtatcagactcagccgtgtac

SEQ ID NO: 228 - DNA, 25 bp, Artificial Sequence
  Primer
gccacaataaacatacaggaaaagc

SEQ ID NO: 229 - DNA, 48 bp, Artificial Sequence
  Primer
atttcaggtgtcgtgaagcggccgcgccaccatgagcatcggcctcct

SEQ ID NO: 230 - DNA, 48 bp, Artificial Sequence; identical to SEQ ID NO: 229
  Primer

SEQ ID NO: 231 - DNA, 48 bp, Artificial Sequence
  Primer
atttcaggtgtcgtgaagcggccgcgccaccatggactcctggacctt

SEQ ID NO: 232 - DNA, 48 bp, Artificial Sequence
  Primer
atttcaggtgtcgtgaagcggccgcgccaccatgggcaccaggctcct

SEQ ID NO: 233 - DNA, 48 bp, Artificial Sequence
  Primer
atttcaggtgtcgtgaagcggccgcgccaccatgggccccgggctcct

SEQ ID NO: 234 - DNA, 48 bp, Artificial Sequence
  Primer
atttcaggtgtcgtgaagcggccgcgccaccatgggctccaggctgct

SEQ ID NO: 235 - DNA, 81 bp, Artificial Sequence
  Primer
tctccagcctgcttcagcaggctgaagttagtagctccgcttccgctccgtttccgccggaaatcctttctcttgaccatg

SEQ ID NO: 236 - DNA, 71 bp, Artificial Sequence
  Primer
tcagcctgctgaagcaggctggagacgtggaggagaaccctggacctatggagaagaatcctttggcagcc

SEQ ID NO: 237 - DNA, 71 bp, Artificial Sequence; identical to SEQ ID NO: 236
  Primer

SEQ ID NO: 238 - DNA, 71 bp, Artificial Sequence
  Primer
tcagcctgctgaagcaggctggagacgtggaggagaaccctggacctatgatgaaatccttgagagtttta

SEQ ID NO: 239 - DNA, 71 bp, Artificial Sequence; identical to SEQ ID NO: 236
  Primer

SEQ ID NO: 240 - DNA, 71 bp, Artificial Sequence
  Primer
tcagcctgctgaagcaggctggagacgtggaggagaaccctggacctatggcatgccctggcttcctgtgg

SEQ ID NO: 241 - DNA, 71 bp, Artificial Sequence
  Primer
tcagcctgctgaagcaggctggagacgtggaggagaaccctggacctatggccatgctcctgggggcatca

SEQ ID NO: 242 - DNA, 45 bp, Artificial Sequence
  Primer
agggatcctctagactcgagctagctcagctggaccacagccgca

SEQ ID NO: 243 - DNA, 25 bp, Artificial Sequence
  Primer
caccgtctctcagctggtacacggc

SEQ ID NO: 244 - DNA, 25 bp, Artificial Sequence
  Primer
aaacgccgtgtaccagctgagagac

SEQ ID NO: 245 - DNA, 25 bp, Artificial Sequence
  Primer
caccgggctcaaacacagcgacctc

SEQ ID NO: 246 - DNA, 25 bp, Artificial Sequence
  Primer
aaacgaggtcgctgtgtttgagccc

SEQ ID NO: 247 - protein, 311 aa, Artificial Sequence
  C22  β aa
MSIGLLCCAALSLLWAGPVNAGVTQTPKFQVLKTGQSMTLQCAQDMNHEYMSWYRQDPGMGLRLIHYSVGAGITDQGEVPNGYNVSRSTTEDFPLRLLSAAPSQTSVYFCASSFATGVGSYGYTFGSGTRLTVVEDLKNVFPPEVAVFEPSEAEISHTQKATLVCLATGFFPDHVELSWWVNGKEVHSGVSTDPQPLKEQPALNDSRYCLSSRLRVSATFWQNPRNHFRCQVQFYGLSENDEWTQDRAKPVTQIVSAEAWGRADCGFTSVSYQQGVLSATILYEILLGKATLYAVLVSALVLMAMVKRKDF

SEQ ID NO: 248 - protein, 309 aa, Artificial Sequence
  C27 β aa
MSIGLLCCAALSLLWAGPVNAGVTQTPKFQVLKTGQSMTLQCAQDMNHEYMSWYRQDPGMGLRLIHYSVGAGITDQGEVPNGYNVSRSTTEDFPLRLLSAAPSQTSVYFCASRPLGVGETQYFGPGTRLLVLEDLKNVFPPEVAVFEPSEAEISHTQKATLVCLATGFFPDHVELSWWVNGKEVHSGVSTDPQPLKEQPALNDSRYCLSSRLRVSATFWQNPRNHFRCQVQFYGLSENDEWTQDRAKPVTQIVSAEAWGRADCGFTSVSYQQGVLSATILYEILLGKATLYAVLVSALVLMAMVKRKDF

SEQ ID NO: 249 - protein, 309 aa, Artificial Sequence
  C29 β aa
MDSWTFCCVSLCILVAKHTDAGVIQSPRHEVTEMGQEVTLRCKPISGHDYLFWYRQTMMRGLELLIYFNNNVPIDDSGMPEDRFSAKMPNASFSTLKIQPSEPRDSAVYFCASSFSLPYEQYFGPGTRLTVTEDLKNVFPPEVAVFEPSEAEISHTQKATLVCLATGFFPDHVELSWWVNGKEVHSGVSTDPQPLKEQPALNDSRYCLSSRLRVSATFWQNPRNHFRCQVQFYGLSENDEWTQDRAKPVTQIVSAEAWGRADCGFTSVSYQQGVLSATILYEILLGKATLYAVLVSALVLMAMVKRKDF

SEQ ID NO: 250 - protein, 310 aa, Artificial Sequence
  C30 β aa
MGTRLLCWVVLGFLGTDHTGAGVSQSPRYKVAKRGQDVALRCDPISGHVSLFWYQQALGQGPEFLTYFQNEAQLDKSGLPSDRFFAERPEGSVSTLKIQRTQQEDSAVYLCASSFYTGQETQYFGPGTRLLVLEDLKNVFPPEVAVFEPSEAEISHTQKATLVCLATGFFPDHVELSWWVNGKEVHSGVSTDPQPLKEQPALNDSRYCLSSRLRVSATFWQNPRNHFRCQVQFYGLSENDEWTQDRAKPVTQIVSAEAWGRADCGFTSVSYQQGVLSATILYEILLGKATLYAVLVSALVLMAMVKRKDF

SEQ ID NO: 251 - protein, 311 aa, Artificial Sequence
  C44 β aa
MGPGLLCWALLCLLGAGLVDAGVTQSPTHLIKTRGQQVTLRCSPKSGHDTVSWYQQALGQGPQFIFQYYEEEERQRGNFPDRFSGHQFPNYSSELNVNALLLGDSALYLCASSFFRGEGNQPQHFGDGTRLSILEDLKNVFPPEVAVFEPSEAEISHTQKATLVCLATGFFPDHVELSWWVNGKEVHSGVSTDPQPLKEQPALNDSRYCLSSRLRVSATFWQNPRNHFRCQVQFYGLSENDEWTQDRAKPVTQIVSAEAWGRADCGFTSVSYQQGVLSATILYEILLGKATLYAVLVSALVLMAMVKRKDF

SEQ ID NO: 252 - protein, 310 aa, Artificial Sequence
  C45 β aa
MGSRLLCWVLLCLLGAGPVKAGVTQTPRYLIKTRGQQVTLSCSPISGHRSVSWYQQTPGQGLQFLFEYFSETQRNKGNFPGRFSGRQFSNSRSEMNVSTLELGDSALYLCASSLAGYKQETQYFGPGTRLLVLEDLKNVFPPEVAVFEPSEAEISHTQKATLVCLATGFFPDHVELSWWVNGKEVHSGVSTDPQPLKEQPALNDSRYCLSSRLRVSATFWQNPRNHFRCQVQFYGLSENDEWTQDRAKPVTQIVSAEAWGRADCGFTSVSYQQGVLSATILYEILLGKATLYAVLVSALVLMAMVKRKDF

SEQ ID NO: 253 - protein, 273 aa, Artificial Sequence
  C22 α aa
MEKNPLAAPLLILWFHLDCVSSILNVEQSPQSLHVQEGDSTNFTCSFPSSNFYALHWYRWETAKSPEALFVMTLNGDEKKKGRISATLNTKEGYSYLYIKGSQPEDSATYLCARNTGNQFYFGTGTSLTVIPNIQNPDPAVYQLRDSKSSDKSVCLFTDFDSQTNVSQSKDSDVYITDKTVLDMRSMDFKSNSAVAWSNKSDFACANAFNNSIIPEDTFFPSPESSCDVKLVEKSFETDTNLNFQNLSVIGFRILLLKVAGFNLLMTLRLWSS

SEQ ID NO: 254 - protein, 272 aa, Artificial Sequence
  C27 α aa
MEKNPLAAPLLILWFHLDCVSSILNVEQSPQSLHVQEGDSTNFTCSFPSSNFYALHWYRWETAKSPEALFVMTLNGDEKKKGRISATLNTKEGYSYLYIKGSQPEDSATYLCASGTYKYIFGTGTRLKVLANIQNPDPAVYQLRDSKSSDKSVCLFTDFDSQTNVSQSKDSDVYITDKTVLDMRSMDFKSNSAVAWSNKSDFACANAFNNSIIPEDTFFPSPESSCDVKLVEKSFETDTNLNFQNLSVIGFRILLLKVAGFNLLMTLRLWSS

SEQ ID NO: 255 - protein, 273 aa, Artificial Sequence
  C29 α aa
MMKSLRVLLVILWLQLSWVWSQQKEVEQDPGPLSVPEGAIVSLNCTYSNSAFQYFMWYRQYSRKGPELLMYTYSSGNKEDGRFTAQVDKSSKYISLFIRDSQPSDSATYLCATFLTGNQFYFGTGTSLTVIPNIQNPDPAVYQLRDSKSSDKSVCLFTDFDSQTNVSQSKDSDVYITDKTVLDMRSMDFKSNSAVAWSNKSDFACANAFNNSIIPEDTFFPSPESSCDVKLVEKSFETDTNLNFQNLSVIGFRILLLKVAGFNLLMTLRLWSS

SEQ ID NO: 256 - protein, 272 aa, Artificial Sequence
  C30 α aa
MEKNPLAAPLLILWFHLDCVSSILNVEQSPQSLHVQEGDSTNFTCSFPSSNFYALHWYRWETAKSPEALFVMTLNGDEKKKGRISATLNTKEGYSYLYIKGSQPEDSATYLCARYGNKLVFGAGTILRVKSYIQNPDPAVYQLRDSKSSDKSVCLFTDFDSQTNVSQSKDSDVYITDKTVLDMRSMDFKSNSAVAWSNKSDFACANAFNNSIIPEDTFFPSPESSCDVKLVEKSFETDTNLNFQNLSVIGFRILLLKVAGFNLLMTLRLWSS

SEQ ID NO: 257 - protein, 278 aa, Artificial Sequence
  C44 α aa
MACPGFLWALVISTCLEFSMAQTVTQSQPEMSVQEAETVTLSCTYDTSESDYYLFWYKQPPSRQMILVIRQEAYKQQNATENRFSVNFQKAAKSFSLKISDSQLGDAAMYFCAYRAFYTGANSKLTFGKGITLSVRPDIQNPDPAVYQLRDSKSSDKSVCLFTDFDSQTNVSQSKDSDVYITDKTVLDMRSMDFKSNSAVAWSNKSDFACANAFNNSIIPEDTFFPSPESSCDVKLVEKSFETDTNLNFQNLSVIGFRILLLKVAGFNLLMTLRLWSS

SEQ ID NO: 258 - protein, 280 aa, Artificial Sequence
  C45 α aa
MAMLLGASVLILWLQPDWVNSQQKNDDQQVKQNSPSLSVQEGRISILNCDYTNSMFDYFLWYKKYPAEGPTFLISISSIKDKNEDGRFTVFLNKSAKHLSLHIVPSQPGDSAVYFCAASAWNTGNQFYFGTGTSLTVIPNIQNPDPAVYQLRDSKSSDKSVCLFTDFDSQTNVSQSKDSDVYITDKTVLDMRSMDFKSNSAVAWSNKSDFACANAFNNSIIPEDTFFPSPESSCDVKLVEKSFETDTNLNFQNLSVIGFRILLLKVAGFNLLMTLRLWSS

SEQ ID NO: 259 - protein, 27 aa, Artificial Sequence
  fp2A aa
RRKRSGSGATNFSLLKQAGDVEENPGP

SEQ ID NO: 260 - DNA, 933 bp, Artificial Sequence
  C22 β NT
atgagcatcggcctcctgtgctgtgcagccttgtctctcctgtgggcaggtccagtgaatgctggtgtcactcagaccccaaaattccaggtcctgaagacaggacagagcatgacactgcagtgtgcccaggatatgaaccatgaatacatgtcctggtatcgacaagacccaggcatggggctgaggctgattcattactcagttggtgctggtatcactgaccaaggagaagtccccaatggctacaatgtctccagatcaaccacagaggatttcccgctcaggctgctgtcggctgctccctcccagacatctgtgtacttctgtgccagcagtttcgcgacaggggtggggagctatggctacaccttcggttcggggaccaggttaaccgttgtagaggacctgaaaaacgtgttcccacccgaggtcgctgtgtttgagccatcagaagcagagatctcccacacccaaaaggccacactggtgtgcctggccacaggcttcttccccgaccacgtggagctgagctggtgggtgaatgggaaggaggtgcacagtggggtcagcacagacccgcagcccctcaaggagcagcccgccctcaatgactccagatactgcctgagcagccgcctgagggtctcggccaccttctggcagaacccccgcaaccacttccgctgtcaagtccagttctacgggctctcggagaatgacgagtggacccaggatagggccaaacccgtcacccagatcgtcagcgccgaggcctggggtagagcagactgtggctttacctcggtgtcctaccagcaaggggtcctgtctgccaccatcctctatgagatcctgctagggaaggccaccctgtatgctgtgctggtcagcgcccttgtgttgatggccatggtcaagagaaaggatttc

SEQ ID NO: 261 - DNA, 927 bp, Artificial Sequence
  C27 β NT
atgagcatcggcctcctgtgctgtgcagccttgtctctcctgtgggcaggtccagtgaatgctggtgtcactcagaccccaaaattccaggtcctgaagacaggacagagcatgacactgcagtgtgcccaggatatgaaccatgaatacatgtcctggtatcgacaagacccaggcatggggctgaggctgattcattactcagttggtgctggtatcactgaccaaggagaagtccccaatggctacaatgtctccagatcaaccacagaggatttcccgctcaggctgctgtcggctgctccctcccagacatctgtgtacttctgtgccagcagaccactgggggtcggcgagacccagtacttcgggccaggcacgcggctcctggtgctcgaggacctgaaaaacgtgttcccacccgaggtcgctgtgtttgagccatcagaagcagagatctcccacacccaaaaggccacactggtgtgcctggccacaggcttcttccccgaccacgtggagctgagctggtgggtgaatgggaaggaggtgcacagtggggtcagcacagacccgcagcccctcaaggagcagcccgccctcaatgactccagatactgcctgagcagccgcctgagggtctcggccaccttctggcagaacccccgcaaccacttccgctgtcaagtccagttctacgggctctcggagaatgacgagtggacccaggatagggccaaacccgtcacccagatcgtcagcgccgaggcctggggtagagcagactgtggctttacctcggtgtcctaccagcaaggggtcctgtctgccaccatcctctatgagatcctgctagggaaggccaccctgtatgctgtgctggtcagcgcccttgtgttgatggccatggtcaagagaaaggatttc

SEQ ID NO: 262 - DNA, 927 bp, Artificial Sequence
  C29 β NT
atggactcctggaccttctgctgtgtgtccctttgcatcctggtagcaaagcacacagatgctggagttatccagtcaccccggcacgaggtgacagagatgggacaagaagtgactctgagatgtaaaccaatttcaggacatgactaccttttctggtacagacagaccatgatgcggggactggagttgctcatttactttaacaacaacgttccgatagatgattcagggatgcccgaggatcgattctcagctaagatgcctaatgcatcattctccactctgaagatccagccctcagaacccagggactcagctgtgtacttctgtgccagcagttttagccttccctacgagcagtacttcgggccgggcaccaggctcacggtcacagaggacctgaaaaacgtgttcccacccgaggtcgctgtgtttgagccatcagaagcagagatctcccacacccaaaaggccacactggtgtgcctggccacaggcttcttccccgaccacgtggagctgagctggtgggtgaatgggaaggaggtgcacagtggggtcagcacagacccgcagcccctcaaggagcagcccgccctcaatgactccagatactgcctgagcagccgcctgagggtctcggccaccttctggcagaacccccgcaaccacttccgctgtcaagtccagttctacgggctctcggagaatgacgagtggacccaggatagggccaaacccgtcacccagatcgtcagcgccgaggcctggggtagagcagactgtggctttacctcggtgtcctaccagcaaggggtcctgtctgccaccatcctctatgagatcctgctagggaaggccaccctgtatgctgtgctggtcagcgcccttgtgttgatggccatggtcaagagaaaggatttc

SEQ ID NO: 263 - DNA, 930 bp, Artificial Sequence
  C30 β NT
atgggcaccaggctcctctgctgggtggtcctgggtttcctagggacagatcacacaggtgctggagtctcccagtcccctaggtacaaagtcgcaaagagaggacaggatgtagctctcaggtgtgatccaatttcgggtcatgtatcccttttttggtaccaacaggccctggggcaggggccagagtttctgacttatttccagaatgaagctcaactagacaaatcggggctgcccagtgatcgcttctttgcagaaaggcctgagggatccgtctccactctgaagatccagcgcacacagcaggaggactccgccgtgtatctctgtgccagcagcttttatacggggcaagagacccagtacttcgggccaggcacgcggctcctggtgctcgaggacctgaaaaacgtgttcccacccgaggtcgctgtgtttgagccatcagaagcagagatctcccacacccaaaaggccacactggtgtgcctggccacaggcttcttccccgaccacgtggagctgagctggtgggtgaatgggaaggaggtgcacagtggggtcagcacagacccgcagcccctcaaggagcagcccgccctcaatgactccagatactgcctgagcagccgcctgagggtctcggccaccttctggcagaacccccgcaaccacttccgctgtcaagtccagttctacgggctctcggagaatgacgagtggacccaggatagggccaaacccgtcacccagatcgtcagcgccgaggcctggggtagagcagactgtggctttacctcggtgtcctaccagcaaggggtcctgtctgccaccatcctctatgagatcctgctagggaaggccaccctgtatgctgtgctggtcagcgcccttgtgttgatggccatggtcaagagaaaggatttc

SEQ ID NO: 264 - DNA, 933 bp, Artificial Sequence
  C44 β NT
atgggccccgggctcctctgctgggcactgctttgtctcctgggagcaggcttagtggacgctggagtcacccaaagtcccacacacctgatcaaaacgagaggacagcaagtgactctgagatgctctcctaagtctgggcatgacactgtgtcctggtaccaacaggccctgggtcaggggccccagtttatctttcagtattatgaggaggaagagagacagagaggcaacttccctgatcgattctcaggtcaccagttccctaactatagctctgagctgaatgtgaacgccttgttgctgggggactcggccctctatctctgtgccagcagctttttccggggcgaggggaatcagccccagcattttggtgatgggactcgactctccatcctagaggacctgaaaaacgtgttcccacccgaggtcgctgtgtttgagccatcagaagcagagatctcccacacccaaaaggccacactggtgtgcctggccacaggcttcttccccgaccacgtggagctgagctggtgggtgaatgggaaggaggtgcacagtggggtcagcacagacccgcagcccctcaaggagcagcccgccctcaatgactccagatactgcctgagcagccgcctgagggtctcggccaccttctggcagaacccccgcaaccacttccgctgtcaagtccagttctacgggctctcggagaatgacgagtggacccaggatagggccaaacccgtcacccagatcgtcagcgccgaggcctggggtagagcagactgtggctttacctcggtgtcctaccagcaaggggtcctgtctgccaccatcctctatgagatcctgctagggaaggccaccctgtatgctgtgctggtcagcgcccttgtgttgatggccatggtcaagagaaaggatttc

SEQ ID NO: 265 - DNA, 930 bp, Artificial Sequence
  C45 β
atgggctccaggctgctctgttgggtgctgctttgtctcctgggagcaggcccagtaaaggctggagtcactcaaactccaagatatctgatcaaaacgagaggacagcaagtgacactgagctgctcccctatctctgggcataggagtgtatcctggtaccaacagaccccaggacagggccttcagttcctctttgaatacttcagtgagacacagagaaacaaaggaaacttccctggtcgattctcagggcgccagttctctaactctcgctctgagatgaatgtgagcaccttggagctgggggactcggccctttatctttgcgccagcagcttggcgggatacaagcaagagacccagtacttcgggccaggcacgcggctcctggtgctcgaggacctgaaaaacgtgttcccacccgaggtcgctgtgtttgagccatcagaagcagagatctcccacacccaaaaggccacactggtgtgcctggccacaggcttcttccccgaccacgtggagctgagctggtgggtgaatgggaaggaggtgcacagtggggtcagcacagacccgcagcccctcaaggagcagcccgccctcaatgactccagatactgcctgagcagccgcctgagggtctcggccaccttctggcagaacccccgcaaccacttccgctgtcaagtccagttctacgggctctcggagaatgacgagtggacccaggatagggccaaacccgtcacccagatcgtcagcgccgaggcctggggtagagcagactgtggctttacctcggtgtcctaccagcaaggggtcctgtctgccaccatcctctatgagatcctgctagggaaggccaccctgtatgctgtgctggtcagcgcccttgtgttgatggccatggtcaagagaaaggatttc

SEQ ID NO: 266 - DNA, 822 bp, Artificial Sequence
  C22 α NT
atggagaagaatcctttggcagccccattactaatcctctggtttcatcttgactgcgtgagcagcatactgaacgtggaacaaagtcctcagtcactgcatgttcaggagggagacagcaccaatttcacctgcagcttcccttccagcaatttttatgccttacactggtacagatgggaaactgcaaaaagccccgaggccttgtttgtaatgactttaaatggggatgaaaagaagaaaggacgaataagtgccactcttaataccaaggagggttacagctatttgtacatcaaaggatcccagcctgaagactcagccacatacctctgtgcccggaacaccggtaaccagttctattttgggacagggacaagtttgacggtcattccaaatatccagaaccctgaccctgccgtgtaccagctgagagactctaaatccagtgacaagtctgtctgcctattcaccgattttgattctcaaacaaatgtgtcacaaagtaaggattctgatgtgtatatcacagacaaaactgtgctagacatgaggtctatggacttcaagagcaacagtgctgtggcctggagcaacaaatctgactttgcatgtgcaaacgccttcaacaacagcattattccagaagacaccttcttccccagcccagaaagttcctgtgatgtcaagctggtcgagaaaagctttgaaacagatacgaacctaaactttcaaaacctgtcagtgattgggttccgaatcctcctcctgaaagtggccgggtttaatctgctcatgacgctgcggctgtggtccagctga

SEQ ID NO: 267 - DNA, 819 bp, Artificial Sequence
  C27 α NT
atggagaagaatcctttggcagccccattactaatcctctggtttcatcttgactgcgtgagcagcatactgaacgtggaacaaagtcctcagtcactgcatgttcaggagggagacagcaccaatttcacctgcagcttcccttccagcaatttttatgccttacactggtacagatgggaaactgcaaaaagccccgaggccttgtttgtaatgactttaaatggggatgaaaagaagaaaggacgaataagtgccactcttaataccaaggagggttacagctatttgtacatcaaaggatcccagcctgaagactcagccacatacctctgtgcttcaggaacctacaaatacatctttggaacaggcaccaggctgaaggttttagcaaatatccagaaccctgaccctgccgtgtaccagctgagagactctaaatccagtgacaagtctgtctgcctattcaccgattttgattctcaaacaaatgtgtcacaaagtaaggattctgatgtgtatatcacagacaaaactgtgctagacatgaggtctatggacttcaagagcaacagtgctgtggcctggagcaacaaatctgactttgcatgtgcaaacgccttcaacaacagcattattccagaagacaccttcttccccagcccagaaagttcctgtgatgtcaagctggtcgagaaaagctttgaaacagatacgaacctaaactttcaaaacctgtcagtgattgggttccgaatcctcctcctgaaagtggccgggtttaatctgctcatgacgctgcggctgtggtccagctga

SEQ ID NO: 268 - DNA, 822 bp, Artificial Sequence
  C29 α   NT
atgatgaaatccttgagagttttactggtgatcctgtggcttcagttaagctgggtttggagccaacagaaggaggtggagcaggatcctggaccactcagtgttccagagggagccattgtttctctcaactgcacttacagcaacagtgcttttcaatacttcatgtggtacagacagtattccagaaaaggccctgagttgctgatgtacacatactccagtggtaacaaagaagatggaaggtttacagcacaggtcgataaatccagcaagtatatctccttgttcatcagagactcacagcccagtgattcagccacctacctctgtgcaacttttttaaccggtaaccagttctattttgggacagggacaagtttgacggtcattccaaatatccagaaccctgaccctgccgtgtaccagctgagagactctaaatccagtgacaagtctgtctgcctattcaccgattttgattctcaaacaaatgtgtcacaaagtaaggattctgatgtgtatatcacagacaaaactgtgctagacatgaggtctatggacttcaagagcaacagtgctgtggcctggagcaacaaatctgactttgcatgtgcaaacgccttcaacaacagcattattccagaagacaccttcttccccagcccagaaagttcctgtgatgtcaagctggtcgagaaaagctttgaaacagatacgaacctaaactttcaaaacctgtcagtgattgggttccgaatcctcctcctgaaagtggccgggtttaatctgctcatgacgctgcggctgtggtccagctga

SEQ ID NO: 269 - DNA, 819 bp, Artificial Sequence
  C30 α NT
atggagaagaatcctttggcagccccattactaatcctctggtttcatcttgactgcgtgagcagcatactgaacgtggaacaaagtcctcagtcactgcatgttcaggagggagacagcaccaatttcacctgcagcttcccttccagcaatttttatgccttacactggtacagatgggaaactgcaaaaagccccgaggccttgtttgtaatgactttaaatggggatgaaaagaagaaaggacgaataagtgccactcttaataccaaggagggttacagctatttgtacatcaaaggatcccagcctgaagactcagccacatacctctgtgcccgatatggaaacaagctggtctttggcgcaggaaccattctgagagtcaagtcctatatccagaaccctgaccctgccgtgtaccagctgagagactctaaatccagtgacaagtctgtctgcctattcaccgattttgattctcaaacaaatgtgtcacaaagtaaggattctgatgtgtatatcacagacaaaactgtgctagacatgaggtctatggacttcaagagcaacagtgctgtggcctggagcaacaaatctgactttgcatgtgcaaacgccttcaacaacagcattattccagaagacaccttcttccccagcccagaaagttcctgtgatgtcaagctggtcgagaaaagctttgaaacagatacgaacctaaactttcaaaacctgtcagtgattgggttccgaatcctcctcctgaaagtggccgggtttaatctgctcatgacgctgcggctgtggtccagctga

SEQ ID NO: 270 - DNA, 837 bp, Artificial Sequence
  C44 α NT
atggcatgccctggcttcctgtgggcacttgtgatctccacctgtcttgaatttagcatggctcagacagtcactcagtctcaaccagagatgtctgtgcaggaggcagagaccgtgaccctgagctgcacatatgacaccagtgagagtgattattatttattctggtacaagcagcctcccagcaggcagatgattctcgttattcgccaagaagcttataagcaacagaatgcaacagagaatcgtttctctgtgaacttccagaaagcagccaaatccttcagtctcaagatctcagactcacagctgggggatgccgcgatgtatttctgtgcttatagggccttttatactggagccaatagtaagctgacatttggaaaaggaataactctgagtgttagaccagatatccagaaccctgaccctgccgtgtaccagctgagagactctaaatccagtgacaagtctgtctgcctattcaccgattttgattctcaaacaaatgtgtcacaaagtaaggattctgatgtgtatatcacagacaaaactgtgctagacatgaggtctatggacttcaagagcaacagtgctgtggcctggagcaacaaatctgactttgcatgtgcaaacgccttcaacaacagcattattccagaagacaccttcttccccagcccagaaagttcctgtgatgtcaagctggtcgagaaaagctttgaaacagatacgaacctaaactttcaaaacctgtcagtgattgggttccgaatcctcctcctgaaagtggccgggtttaatctgctcatgacgctgcggctgtggtccagctga

SEQ ID NO: 271 - DNA, 843 bp, Artificial Sequence
  C45 α NT
atggccatgctcctgggggcatcagtgctgattctgtggcttcagccagactgggtaaacagtcaacagaagaatgatgaccagcaagttaagcaaaattcaccatccctgagcgtccaggaaggaagaatttctattctgaactgtgactatactaacagcatgtttgattatttcctatggtacaaaaaataccctgctgaaggtcctacattcctgatatctataagttccattaaggataaaaatgaagatggaagattcactgttttcttaaacaaaagtgccaagcacctctctctgcacattgtgccctcccagcctggagactctgcagtgtacttctgtgcagcaagcgcgtggaacaccggtaaccagttctattttgggacagggacaagtttgacggtcattccaaatatccagaaccctgaccctgccgtgtaccagctgagagactctaaatccagtgacaagtctgtctgcctattcaccgattttgattctcaaacaaatgtgtcacaaagtaaggattctgatgtgtatatcacagacaaaactgtgctagacatgaggtctatggacttcaagagcaacagtgctgtggcctggagcaacaaatctgactttgcatgtgcaaacgccttcaacaacagcattattccagaagacaccttcttccccagcccagaaagttcctgtgatgtcaagctggtcgagaaaagctttgaaacagatacgaacctaaactttcaaaacctgtcagtgattgggttccgaatcctcctcctgaaagtggccgggtttaatctgctcatgacgctgcggctgtggtccagctga

SEQ ID NO: 272 - DNA, 81 bp, Artificial Sequence
  fp2A NT
cggcggaaacggagcggaagcggagctactaacttcagcctgctgaagcaggctggagacgtggaggagaaccctggacct

SEQ ID NO: 273 - protein, 612 aa, Artificial Sequence
  C2 AA
MGPQLLGYVVLCLLGAGPLEAQVTQNPRYLITVTGKKLTVTCSQNMNHEYMSWYRQDPGLGLRQIYYSMNVEVTDKGDVPEGYKVSRKEKRNFPLILESPSPNQTSLYFCASSPTLGTGAETQYFGPGTRLLVLEDLKNVFPPEVAVFEPSEAEISHTQKATLVCLATGFFPDHVELSWWVNGKEVHSGVSTDPQPLKEQPALNDSRYCLSSRLRVSATFWQNPRNHFRCQVQFYGLSENDEWTQDRAKPVTQIVSAEAWGRADCGFTSVSYQQGVLSATILYEILLGKATLYAVLVSALVLMAMVKRKDFRRKRSGSGATNFSLLKQAGDVEENPGPMMEKNPLAAPLLILWFHLDCVSSILNVEQSPQSLHVQEGDSTNFTCSFPSSNFYALHWYRWETAKSPEALFVMTLNGDEKKKGRISATLNTKEGYSYLYIKGSQPEDSATYLCASPYFNKFYFGSGTKLNVKPNIQNPDPAVYQLRDSKSSDKSVCLFTDFDSQTNVSQSKDSDVYITDKTVLDMRSMDFKSNSAVAWSNKSDFACANAFNNSIIPEDTFFPSPESSCDVKLVEKSFETDTNLNFQNLSVIGFRILLLKVAGFNLLMTLRLWSS

SEQ ID NO: 274 - DNA, 1839 bp, Artificial Sequence
  C2 NT
atgggcccccagctccttggctatgtggtcctttgccttctaggagcaggccccctggaagcccaagtgacccagaacccaagatacctcatcacagtgactggaaagaagttaacagtgacttgttctcagaatatgaaccatgagtatatgtcctggtatcgacaagacccagggctgggcttaaggcagatctactattcaatgaatgttgaggtgactgataagggagatgttcctgaagggtacaaagtctctcgaaaagagaagaggaatttccccctgatcctggagtcgcccagccccaaccagacctctctgtacttctgtgccagcagccctaccctagggacaggggccgagacccagtacttcgggccaggcacgcggctcctggtgctcgaggacctgaaaaacgtgttcccacccgaggtcgctgtgtttgagccatcagaagcagagatctcccacacccaaaaggccacactggtgtgcctggccacaggcttcttccccgaccacgtggagctgagctggtgggtgaatgggaaggaggtgcacagtggggtcagcacagacccgcagcccctcaaggagcagcccgccctcaatgactccagatactgcctgagcagccgcctgagggtctcggccaccttctggcagaacccccgcaaccacttccgctgtcaagtccagttctacgggctctcggagaatgacgagtggacccaggatagggccaaacccgtcacccagatcgtcagcgccgaggcctggggtagagcagactgtggctttacctcggtgtcctaccagcaaggggtcctgtctgccaccatcctctatgagatcctgctagggaaggccaccctgtatgctgtgctggtcagcgcccttgtgttgatggccatggtcaagagaaaggatttccggcggaaacggagcggaagcggagctactaacttcagcctgctgaagcaggctggagacgtggaggagaaccctggacctatgatggagaagaatcctttggcagccccattactaatcctctggtttcatcttgactgcgtgagcagcatactgaacgtggaacaaagtcctcagtcactgcatgttcaggagggagacagcaccaatttcacctgcagcttcccttccagcaatttttatgccttacactggtacagatgggaaactgcaaaaagccccgaggccttgtttgtaatgactttaaatggggatgaaaagaagaaaggacgaataagtgccactcttaataccaaggagggttacagctatttgtacatcaaaggatcccagcctgaagactcagccacatacctctgtgcctcaccgtacttcaacaaattttactttggatctgggaccaaactcaatgtaaaaccaaatatccagaaccctgaccctgccgtgtaccagctgagagactctaaatccagtgacaagtctgtctgcctattcaccgattttgattctcaaacaaatgtgtcacaaagtaaggattctgatgtgtatatcacagacaaaactgtgctagacatgaggtctatggacttcaagagcaacagtgctgtggcctggagcaacaaatctgactttgcatgtgcaaacgccttcaacaacagcattattccagaagacaccttcttccccagcccagaaagttcctgtgatgtcaagctggtcgagaaaagctttgaaacagatacgaacctaaactttcaaaacctgtcagtgattgggttccgaatcctcctcctgaaagtggccgggtttaatctgctcatgacgctgcggctgtggtccagctga

SEQ ID NO: 275 - protein, 311 aa, Artificial Sequence
  C2 β AA
MGPQLLGYVVLCLLGAGPLEAQVTQNPRYLITVTGKKLTVTCSQNMNHEYMSWYRQDPGLGLRQIYYSMNVEVTDKGDVPEGYKVSRKEKRNFPLILESPSPNQTSLYFCASSPTLGTGAETQYFGPGTRLLVLEDLKNVFPPEVAVFEPSEAEISHTQKATLVCLATGFFPDHVELSWWVNGKEVHSGVSTDPQPLKEQPALNDSRYCLSSRLRVSATFWQNPRNHFRCQVQFYGLSENDEWTQDRAKPVTQIVSAEAWGRADCGFTSVSYQQGVLSATILYEILLGKATLYAVLVSALVLMAMVKRKDF

SEQ ID NO: 276 - protein, 274 aa, Artificial Sequence
  C2 α AA
MMEKNPLAAPLLILWFHLDCVSSILNVEQSPQSLHVQEGDSTNFTCSFPSSNFYALHWYRWETAKSPEALFVMTLNGDEKKKGRISATLNTKEGYSYLYIKGSQPEDSATYLCASPYFNKFYFGSGTKLNVKPNIQNPDPAVYQLRDSKSSDKSVCLFTDFDSQTNVSQSKDSDVYITDKTVLDMRSMDFKSNSAVAWSNKSDFACANAFNNSIIPEDTFFPSPESSCDVKLVEKSFETDTNLNFQNLSVIGFRILLLKVAGFNLLMTLRLWSS

SEQ ID NO: 277 - DNA, 933 bp, Artificial Sequence
  C2 β NT
atgggcccccagctccttggctatgtggtcctttgccttctaggagcaggccccctggaagcccaagtgacccagaacccaagatacctcatcacagtgactggaaagaagttaacagtgacttgttctcagaatatgaaccatgagtatatgtcctggtatcgacaagacccagggctgggcttaaggcagatctactattcaatgaatgttgaggtgactgataagggagatgttcctgaagggtacaaagtctctcgaaaagagaagaggaatttccccctgatcctggagtcgcccagccccaaccagacctctctgtacttctgtgccagcagccctaccctagggacaggggccgagacccagtacttcgggccaggcacgcggctcctggtgctcgaggacctgaaaaacgtgttcccacccgaggtcgctgtgtttgagccatcagaagcagagatctcccacacccaaaaggccacactggtgtgcctggccacaggcttcttccccgaccacgtggagctgagctggtgggtgaatgggaaggaggtgcacagtggggtcagcacagacccgcagcccctcaaggagcagcccgccctcaatgactccagatactgcctgagcagccgcctgagggtctcggccaccttctggcagaacccccgcaaccacttccgctgtcaagtccagttctacgggctctcggagaatgacgagtggacccaggatagggccaaacccgtcacccagatcgtcagcgccgaggcctggggtagagcagactgtggctttacctcggtgtcctaccagcaaggggtcctgtctgccaccatcctctatgagatcctgctagggaaggccaccctgtatgctgtgctggtcagcgcccttgtgttgatggccatggtcaagagaaaggatttc

SEQ ID NO: 278 - DNA, 825 bp, Artificial Sequence
  C2 α NT
atgatggagaagaatcctttggcagccccattactaatcctctggtttcatcttgactgcgtgagcagcatactgaacgtggaacaaagtcctcagtcactgcatgttcaggagggagacagcaccaatttcacctgcagcttcccttccagcaatttttatgccttacactggtacagatgggaaactgcaaaaagccccgaggccttgtttgtaatgactttaaatggggatgaaaagaagaaaggacgaataagtgccactcttaataccaaggagggttacagctatttgtacatcaaaggatcccagcctgaagactcagccacatacctctgtgcctcaccgtacttcaacaaattttactttggatctgggaccaaactcaatgtaaaaccaaatatccagaaccctgaccctgccgtgtaccagctgagagactctaaatccagtgacaagtctgtctgcctattcaccgattttgattctcaaacaaatgtgtcacaaagtaaggattctgatgtgtatatcacagacaaaactgtgctagacatgaggtctatggacttcaagagcaacagtgctgtggcctggagcaacaaatctgactttgcatgtgcaaacgccttcaacaacagcattattccagaagacaccttcttccccagcccagaaagttcctgtgatgtcaagctggtcgagaaaagctttgaaacagatacgaacctaaactttcaaaacctgtcagtgattgggttccgaatcctcctcctgaaagtggccgggtttaatctgctcatgacgctgcggctgtggtccagctga

SEQ ID NO: 279 - DNA, 48 bp, Artificial Sequence
  Primer
atttcaggtgtcgtgaagcggccgcgccaccatgggcccccagctcct

SEQ ID NO: 280 - DNA, 71 bp, Artificial Sequence
  Primer
tcagcctgctgaagcaggctggagacgtggaggagaaccctggacctatgatggagaagaatcctttggca

SEQ ID NO: 281 - protein, 9 aa, Artificial Sequence
  CDR
ASPYFNKFY

SEQ ID NO: 282 - protein, 6 aa, Artificial Sequence
  CDR
SMNVEV

SEQ ID NO: 283 - protein, 14 aa, Artificial Sequence
  CDR
ASSPTLGTGAETQY